European Patent Application EP 4 477 266 A2, published December 18, 2024. Title: METHODS AND MATERIALS FOR TREATING PROTEINOPATHIES. Applicant: Mayo Foundation for Medical Education and Research. Application EP. The sequence listing filed with the application follows.

SEQUENCE LISTING (80 sequences)

SEQ ID NO: 1 - protein, 876 aa, Homo sapiens
MELITILEKTVSPDRLELEAAQKFLERAAVENLPTFLVELSRVLANPGNSQVARVAAGLQIKNSLTSKDPDIKAQYQQRWLAIDANARREVKNYVLQTLGTETYRPSSASQCVAGIACAEIPVNQWPELIPQLVANVTNPNSTEHMKESTLEAIGYICQDIDPEQLQDKSNEILTAIIQGMRKEEPSNNVKLAATNALLNSLEFTKANFDKESERHFIMQVVCEATQCPDTRVRVAALQNLVKIMSLYYQYMETYMGPALFAITIEAMKSDIDEVALQGIEFWSNVCDEEMDLAIEASEAAEQGRPPEHTSKFYAKGALQYLVPILTQTLTKQDENDDDDDWNPCKAAGVCLMLLATCCEDDIVPHVLPFIKEHIKNPDWRYRDAAVMAFGCILEGPEPSQLKPLVIQAMPTLIELMKDPSVVVRDTAAWTVGRICELLPEAAINDVYLAPLLQCLIEGLSAEPRVASNVCWAFSSLAEAAYEAADVADDQEEPATYCLSSSFELIVQKLLETTDRPDGHQNNLRSSAYESLMEIVKNSAKDCYPAVQKTTLVIMERLQQVLQMESHIQSTSDRIQFNDLQSLLCATLQNVLRKVQHQDALQISDVVMASLLRMFQSTAGSGGVQEDALMAVSTLVEVLGGEFLKYMEAFKPFLGIGLKNYAEYQVCLAAVGLVGDLCRALQSNIIPFCDEVMQLLLENLGNENVHRSVKPQILSVFGDIALAIGGEFKKYLEVVLNTLQQASQAQVDKSDYDMVDYLNELRESCLEAYTGIVQGLKGDQENVHPDVMLVQPRVEFILSFIDHIAGDEDHTDGVVACAAGLIGDLCTAFGKDVLKLVEARPMIHELLTEGRRSKTNKAKTLATWATKELRKLKNQA

SEQ ID NO: 2 - DNA, 2631 bp, Homo sapiens
  source 1..2631: mol_type = other DNA
atggagctgatcaccattctcgagaagaccgtgtctcccgatcggctggagctggaagcggcgcagaagttcctggagcgtgcggccgtggagaacctgcccactttccttgtggaactgtccagagtgctggcaaatccaggaaacagtcaggttgccagagttgcagctggtctacaaatcaagaactctttgacatctaaagatccagatatcaaggcacaatatcagcagaggtggcttgctattgatgctaatgctcgacgagaagtcaagaactatgttttgcagacattgggtacagaaacttaccggcctagttctgcctcacagtgtgtggctggtattgcttgtgcagagatcccagtaaaccagtggccagaactcattcctcagctggtggccaatgtcacaaaccccaacagcacagagcacatgaaggagtcgacattggaagccatcggttatatttgccaagatatagacccagagcagctacaagataaatccaatgagattctgactgccataatccaggggatgaggaaagaagagcctagtaataatgtgaagctagctgctacgaatgcactcctgaactcattggagttcaccaaagcaaactttgataaagagtctgaaaggcactttattatgcaggtggtctgtgaagccacacagtgtccagatacgagggtacgagtggctgctttacagaatctggtgaagataatgtccttatattatcagtacatggagacatatatgggtcctgctctttttgcaatcacaatcgaagcaatgaaaagtgacattgatgaggtggctttacaagggatagaattctggtccaatgtctgtgatgaggaaatggatttggccattgaagcttcagaggcagcagaacaaggacggccccctgagcacaccagcaagttttatgcgaagggagcactacagtatctggttccaatcctcacacagacactaactaaacaggacgaaaatgatgatgacgatgactggaacccctgcaaagcagcaggggtgtgcctcatgcttctggccacctgctgtgaagatgacattgtcccacatgtcctccccttcattaaagaacacatcaagaacccagattggcggtaccgggatgcagcagtgatggcttttggttgtatcttggaaggaccagagcccagtcagctcaaaccactagttatacaggctatgcccaccctaatagaattaatgaaagaccccagtgtagttgttcgagatacagctgcatggactgtaggcagaatttgtgagctgcttcctgaagctgccatcaatgatgtctacttggctcccctgctacagtgtctgattgagggtctcagtgctgaacccagagtggcttcaaatgtgtgctgggctttctccagtctggctgaagctgcttatgaagctgcagacgttgctgatgatcaggaagaaccagctacttactgcttatcttcttcatttgaactcatagttcagaagctcctagagactacagacagacctgatggacaccagaacaacctgaggagttctgcatatgaatctctgatggaaattgtgaaaaacagtgccaaggattgttatcctgctgtccagaaaacgactttggtcatcatggaacgactgcaacaggttcttcagatggagtcacatatccagagcacatccgatagaatccagttcaatgaccttcagtctttactctgtgcaactcttcagaatgttcttcggaaagtgcaacatcaagatgctttgcagatctctgatgtggttatggcctccctgttaaggatgttccaaagcacagctgggtctgggggagtacaagaggatgccctgatggcagttagcacactggtggaagtgttgggtggtgaattcctcaagtacatggaggcctttaaacccttcctgggcattggattaaaaaattatgctgaataccaggtttgtttggcagctgtgggcttagtgggagacttgtgccgtgccctgcaatccaacatcatacctttctgtgacgaggtgatgcagctgcttctggaaaatttggggaatgagaacgtccacaggtctgtgaagccgcagattctgtcagtgtttggtgatattgcccttgctattggaggagagtttaaaaaatacttagaggttgtattgaatactcttcagcaggcctcccaagcccaggtggacaagtcagactatgacatggtggattatctgaatgagctaagggaaagctgcttggaagcctatactggaatcgtccagggattaaagggggatcaggagaacgtacacccggatgtgatgctggtacaacccagagtagaatttattctgtctttcattgaccacattgctggagatgaggatcacacagatggagtagtagcttgtgctgctggactaataggggacttatgtacagcatttgggaaggatgtactgaaattagtagaagctaggccaatgatccatgaattgttaactgaagggcggagatcgaagactaacaaagcaaaaacccttgctacatgggcaacaaaagaactgaggaaactgaagaaccaagcttaa

SEQ ID NO: 3 - protein, 887 aa, Homo sapiens
MDWQPDEQGLQQVLQLLKDSQSPNTATQRIVQDKLKQLNQFPDFNNYLIFVLTRLKSEDEPTRSLSGLILKNNVKAHYQSFPPPVADFIKQECLNNIGDASSLIRATIGILITTIASKGELQMWPELLPQLCNLLNSEDYNTCEGAFGALQKICEDSSELLDSDALNRPLNIMIPKFLQFFKHCSPKIRSHAIACVNQFIMDRAQALMDNIDTFIEHLFALAVDDDPEVRKNVCRALVMLLEVRIDRLIPHMHSIIQYMLQRTQDHDENVALEACEFWLTLAEQPICKEVLASHLVQLIPILVNGMKYSEIDIILLKGDVEEDEAVPDSEQDIKPRFHKSRTVTLPHEAERPDGSEDAEDDDDDDALSDWNLRKCSAAALDVLANVFREELLPHLLPLLKGLLFHPEWVVKESGILVLGAIAEGCMQGMVPYLPELIPHLIQCLSDKKALVRSIACWTLSRYAHWVVSQPPDMHLKPLMTELLKRILDGNKRVQEAACSAFATLEEEACTELVPYLSYILDTLVFAFGKYQHKNLLILYDAIGTLADSVGHHLNQPEYIQKLMPPLIQKWNELKDEDKDLFPLLECLSSVATALQSGFLPYCEPVYQRCVTLVQKTLAQAMMYTQHPEQYEAPDKDFMIVALDLLSGLAEGLGGHVEQLVARSNIMTLLFQCMQDSMPEVRQSSFALLGDLTKACFIHVKPCIAEFMPILGTNLNPEFISVCNNATWAIGEICMQMGAEMQPYVQMVLNNLVEIINRPNTPKTLLENTAITIGRLGYVCPQEVAPMLQQFIRPWCTSLRNIRDNEEKDSAFRGICMMIGVNPGGVVQDFIFFCDAVASWVSPKDDLRDMFYKILHGFKDQVGEDNWQQFSEQFPPLLKERLAAFYGV

SEQ ID NO: 4 - DNA, 2664 bp, Homo sapiens
  source 1..2664: mol_type = other DNA
atggactggcagccagacgagcagggcctgcagcaggtcctgcagctgctcaaagactcacagtcgcccaacacagccactcagcgcatcgtgcaggataaactcaaacaactcaatcagtttcctgacttcaacaactacctgattttcgtcctgaccagactcaagtcagaagatgagccaacgcgctctctcagtggcctcatcctcaagaacaacgtgaaggcacactatcagagcttcccaccccctgtggcagacttcatcaaacaggagtgtctcaacaacattggcgatgcctcctcgctcatccgagccaccattggcattctcatcaccaccatcgcttccaagggtgagctgcagatgtggcccgagctgctgccccagctctgcaacctgcttaactcggaggattacaacacttgtgagggagcctttggagccctgcagaagatctgtgaagactcatcagagcttctggacagtgacgccctcaacaggcccctcaacatcatgatccccaagttcctgcagttcttcaagcactgcagtcccaagatccggtcccacgccatcgcctgcgtgaaccagttcatcatggaccgggcccaggcgctgatggacaatattgacaccttcatcgagcacctatttgccctggctgtggatgatgaccccgaggtgcggaagaatgtgtgccgtgccctggtgatgcttctggaagtgcggattgacaggctcatcccccacatgcacagcatcatccagtacatgctgcagaggacccaggaccatgatgagaacgttgcccttgaggcctgtgagttctggctgacgctggccgagcagcccatctgcaaggaagtcctggcctcccatctggtccagttgatccccatcttggtgaatgggatgaagtactcggaaattgacatcatcctgctcaagggggatgtggaggaggatgaggctgtccccgacagtgagcaggacatcaagccacgcttccacaagtcacgcacggtcacactgccccacgaggctgagcggcctgatggctccgaggacgcggaggatgacgatgatgatgatgctctgtccgactggaatttgaggaagtgctcagcggctgcactggacgtcctcgccaatgtcttccgggaggaactgctgccccacctactcccactactcaaaggcctcctcttccaccccgagtgggtggtcaaggagtcgggcatcctggtgctgggcgccattgctgagggctgcatgcagggcatggtgccctacctgcctgagctgatcccgcacctgatccagtgcctgtcggataagaaggccttggtccgctccatcgcctgctggacgctgagccgctatgcccactgggtggtcagccagccacccgacatgcacctcaagcccctgatgacagagctgctcaaacgcatcctggatggcaacaagagggtacaggaggcggcctgcagtgcttttgccaccctggaggaagaggcctgcacggagctggtgccctacctcagctacatcctggacacccttgtctttgcctttgggaaataccagcacaagaacctgctcatcctctatgacgccattggcaccctggccgactctgtaggccaccacctcaaccagccggaatacatccagaagctgatgcccccactgatccagaagtggaatgagctcaaggacgaagacaaggacctcttccccctgctggagtgtctgtcatcggtggccaccgccctgcagagtggcttcctgccttactgtgagcccgtctaccagcgctgtgtcaccctggtgcagaagacactggctcaggccatgatgtacacccagcaccctgagcagtatgaggctcccgacaaggacttcatgatcgtagcactggatctgctcagcggcctggccgagggcctgggtggtcacgtggagcagctggtggcccgcagcaacatcatgacattgctgttccagtgcatgcaggactcgatgcctgaggtccggcagagctcctttgccctcctgggagacctcaccaaagcctgcttcatccatgtcaagccctgtatcgccgagttcatgcccattctgggcaccaacctgaacccagagttcatctccgtctgcaacaacgccacctgggccattggtgaaatctgcatgcagatgggggcagagatgcagccttatgtgcagatggtcctcaacaacctggtggaaatcattaaccgacccaacacacccaagacactgctggaaaacacagccatcaccatcggccgcttgggctacgtgtgcccccaggaggtggcacccatgctgcagcagttcatccggccttggtgcacgtccctcaggaacatcagggacaacgaggagaaggactcagccttccgcggcatctgcatgatgatcggtgtcaacccggggggcgttgtgcaggactttattttcttctgcgatgctgtagcctcctgggtgagcccgaaggatgaccttcgggacatgttttataagattctccacggcttcaaagaccaagttggggaagataactggcagcagttctctgagcaattcccgccgctgctcaaggagaggctggcggctttctatggggtctag

SEQ ID NO: 5 - protein, 963 aa, Homo sapiens
MERREEQPGAAGAGAAPALDFTVENVEKALHQLYYDPNIENKNLAQKWLMQAQVSPQAWHFSWQLLQPDKVPEIQYFGASALHIKISRYWSDIPTDQYESLKAQLFTQITRFASGSKIVLTRLCVALASLALSMMPDAWPCAVADMVRLFQAEDSPVDGQGRCLALLELLTVLPEEFQTSRLPQYRKGLVRTSLAVECGAVFPLLEQLLQQPSSPSCVRQKVLKCFSSWVQLEVPLQDCEALIQAAFAALQDSELFDSSVEAIVNAISQPDAQRYVNTLLKLIPLVLGLQEQLRQAVQNGDMETSHGICRIAVALGENHSRALLDQVEHWQSFLALVNMIMFCTGIPGHYPVNETTSSLTLTFWYTLQDDILSFEAEKQAVYQQVYRPVYFQLVDVLLHKAQFPSDEEYGFWSSDEKEQFRIYRVDISDTLMYVYEMLGAELLSNLYDKLGRLLTSSEEPYSWQHTEALLYGFQSIAETIDVNYSDVVPGLIGLIPRISISNVQLADTVMFTIGALSEWLADHPVMINSVLPLVLHALGNPELSVSSVSTLKKICRECKYDLPPYAANIVAVSQDVLMKQIHKTSQCMWLMQALGFLLSALQVEEILKNLHSLISPYIQQLEKLAEEIPNPSNKLAIVHILGLLSNLFTTLDISHHEDDHEGPELRKLPVPQGPNPVVVVLQQVFQLIQKVLSKWLNDAQVVEAVCAIFEKSVKTLLDDFAPMVPQLCEMLGRMYSTIPQASALDLTRQLVHIFAHEPAHFPPIEALFLLVTSVTLTLFQQGPRDHPDIVDSFMQLLAQALKRKPDLFLCERLDVKSVFQCAVLALKFPEAPTVKASCGFFTELLPRCGEVESVGKVVQEDGRMLLIAVLEAIGGQASRSLMDCFADILFALNKHCFSLLSMWIKEALQPPGFPSARLSPEQKDTFSQQILRERVNKRRVKEMVKEFTLLCRGLHGTDYTADY

SEQ ID NO: 6 - DNA, 2892 bp, Homo sapiens
  source 1..2892: mol_type = other DNA
atggagcggcgggaggagcagccgggggctgcaggggctggagcagcaccagccttggacttcactgtggagaacgtggagaaggcgctgcaccagctctactatgatcccaacattgagaataagaacctggctcagaagtggctgatgcaggcccaggtctccccacaggcctggcacttcagctggcagctactgcagcccgacaaggtaccagagatccagtactttggggccagtgctcttcacatcaagatctctcgctactggagtgacatccccactgaccagtatgaaagcctaaaggcacagctcttcacccagatcacccgctttgccagtggctccaagattgtactgactcggctgtgcgtggcactggcctcactggctctcagcatgatgcctgatgcttggccatgtgctgtggcagatatggtacgactcttccaggctgaggactcaccagtggatgggcagggccgctgcctagccctgttagagctgctgacagtgctgcctgaggagttccagaccagtcgcctaccccagtaccgcaaaggcctggtgcggaccagcctggcggtggaatgtggggctgtcttcccgctgctggagcagctgctacagcagcccagctcacccagctgtgtgcgtcagaaggtgctcaagtgtttctccagctgggtgcagctggaggtgccgctgcaggactgtgaggcgctcattcaggctgcctttgctgctctgcaggactcggagctcttcgacagcagtgtggaggccattgtgaatgccatctcacagcctgatgcccagaggtacgtgaacacactcctgaaactcatcccgctggtgctgggtctgcaggaacaactgcggcaggcagtgcagaatggggacatggagacctcccatggcatctgtcgcatcgctgtggccctgggcgagaaccactcccgggccttgctggaccaagtagagcactggcagagtttcctggcactcgtcaacatgattatgttctgcacaggcatccctggccactatcctgtcaatgagaccaccagctccctaaccctcaccttctggtacacactgcaggatgatattctatcctttgaggcagagaagcaggctgtataccagcaggtgtaccggccagtctacttccagctggtggatgtgcttctgcacaaggcccagttcccttctgatgaggaatatggattctggtcctcagacgagaaggagcagttccgaatttacagggtggacatctcagacacgctcatgtatgtctatgagatgttgggggccgagctgctcagcaacctctatgacaagctgggtcgtttgctcaccagctcagaggagccctactcctggcagcacacagaggccctcctctacggcttccaatccatcgcagagaccattgacgtcaactattctgatgtggtgcctgggctcattggcctcatcccacggatcagcatcagcaacgtgcagctggcagacactgtcatgttcaccattggagctctgtctgaatggctggctgaccaccccgtcatgatcaacagtgttctgcccttggtactgcatgccctaggcaatcctgagctgtctgtctcttctgtgtccaccctcaagaagatctgccgagagtgcaagtatgacctgcctccctatgctgccaacattgtggctgtgtcccaggatgtgctgatgaaacagatccacaagacaagccagtgcatgtggctgatgcaggcgctgggcttcctgctgtcagctcttcaagtggaggagatccttaagaacctgcactcgcttatctcaccctatatccagcaactggagaagctggcagaggagatacccaatccctccaacaagctggccattgttcacatcttggggcttctctccaacctcttcaccacactggacatcagtcatcatgaggatgatcatgaaggccctgagcttcggaagctgccagtgccacagggacccaaccccgtggtggtggtgctgcagcaggtcttccagcttatccagaaggtgctgagcaaatggttgaatgatgcccaggttgtggaggcggtgtgcgctatctttgagaagtctgttaagacgctgctggatgactttgcccccatggtgccacagctgtgtgagatgctgggtcggatgtacagcaccatcccccaggcctctgctcttgacctcactcgacagctggtccacatctttgctcatgagcctgcccactttcccccaattgaggccctcttcctgctcgtcacctccgtcacactcactctcttccagcaagggcccagggatcatcctgatattgttgattcatttatgcaactcctggcacaggctctgaagcggaagccagatttgttcctgtgtgaacgattggatgtcaaatctgtgttccagtgtgctgtgctggccctcaagttccctgaggcacctactgtcaaggcctcctgtggcttctttacagagctgctgcctcggtgtggggaagtagagtctgtgggaaaggtggtacaggaagacggtcgtatgctgctcatagcagtgctggaggccattgggggccaggcctcccgcagcctcatggactgctttgccgatatcctgttcgccctgaacaagcactgcttcagcctcctgagcatgtggatcaaggaggccctgcagccacctggtttcccctctgcccgcctcagccctgaacagaaggataccttcagccagcagatccttcgcgagcgagtgaacaagaggcgggtgaaggagatggtgaaggagttcacactgctgtgccggggtctccatggcacagattacacagctgactactga

SEQ ID NO: 7 - protein, 397 aa, synthetic construct
  REGION 1..397: note = KPNB1 polypeptide fragment
MELITILEKTVSPDRLELEAAQKFLERAAVENLPTFLVELSRVLANPGNSQVARVAAGLQIKNSLTSKDPDIKAQYQQRWLAIDANARREVKNYVLQTLGTETYRPSSASQCVAGIACAEIPVNQWPELIPQLVANVTNPNSTEHMKESTLEAIGYICQDIDPEQLQDKSNEILTAIIQGMRKEEPSNNVKLAATNALLNSLEFTKANFDKESERHFIMQVVCEATQCPDTRVRVAALQNLVKIMSLYYQYMETYMGPALFAITIEAMKSDIDEVALQGIEFWSNVCDEEMDLAIEASEAAEQGRPPEHTSKFYAKGALQYLVPILTQTLTKQDENDDDDDWNPCKAAGVCLMLLATCCEDDIVPHVLPFIKEHIKNPDWRYRDAAVMAFGCILEGP

SEQ ID NO: 8 - protein, 361 aa, synthetic construct
  REGION 1..361: note = KPNB1 polypeptide fragment
MELITILEKTVSPDRLELEAAQKFLERAAVENLPTFLVELSRVLANPGNSQVARVAAGLQIKNSLTSKDPDIKAQYQQRWLAIDANARREVKNYVLQTLGTETYRPSSASQCVAGIACAEIPVNQWPELIPQLVANVTNPNSTEHMKESTLEAIGYICQDIDPEQLQDKSNEILTAIIQGMRKEEPSNNVKLAATNALLNSLEFTKANFDKESERHFIMQVVCEATQCPDTRVRVAALQNLVKIMSLYYQYMETYMGPALFAITIEAMKSDIDEVALQGIEFWSNVCDEEMDLAIEASEAAEQGRPPEHTSKFYAKGALQYLVPILTQTLTKQDENDDDDDWNPCKAAGVCLMLLATCCED

SEQ ID NO: 9 - protein, 307 aa, synthetic construct
  REGION 1..307: note = KPNB1 polypeptide fragment
MELITILEKTVSPDRLELEAAQKFLERAAVENLPTFLVELSRVLANPGNSQVARVAAGLQIKNSLTSKDPDIKAQYQQRWLAIDANARREVKNYVLQTLGTETYRPSSASQCVAGIACAEIPVNQWPELIPQLVANVTNPNSTEHMKESTLEAIGYICQDIDPEQLQDKSNEILTAIIQGMRKEEPSNNVKLAATNALLNSLEFTKANFDKESERHFIMQVVCEATQCPDTRVRVAALQNLVKIMSLYYQYMETYMGPALFAITIEAMKSDIDEVALQGIEFWSNVCDEEMDLAIEASEAAEQGRPP

SEQ ID NO: 10 - protein, 249 aa, synthetic construct
  REGION 1..249: note = KPNB1 polypeptide fragment
MELITILEKTVSPDRLELEAAQKFLERAAVENLPTFLVELSRVLANPGNSQVARVAAGLQIKNSLTSKDPDIKAQYQQRWLAIDANARREVKNYVLQTLGTETYRPSSASQCVAGIACAEIPVNQWPELIPQLVANVTNPNSTEHMKESTLEAIGYICQDIDPEQLQDKSNEILTAIIQGMRKEEPSNNVKLAATNALLNSLEFTKANFDKESERHFIMQVVCEATQCPDTRVRVAALQNLVKIMSLYY

SEQ ID NO: 11 - protein, 209 aa, synthetic construct
  REGION 1..209: note = KPNB1 polypeptide fragment
MELITILEKTVSPDRLELEAAQKFLERAAVENLPTFLVELSRVLANPGNSQVARVAAGLQIKNSLTSKDPDIKAQYQQRWLAIDANARREVKNYVLQTLGTETYRPSSASQCVAGIACAEIPVNQWPELIPQLVANVTNPNSTEHMKESTLEAIGYICQDIDPEQLQDKSNEILTAIIQGMRKEEPSNNVKLAATNALLNSLEFTKANF

SEQ ID NO: 12 - protein, 167 aa, synthetic construct
  REGION 1..167: note = KPNB1 polypeptide fragment
MELITILEKTVSPDRLELEAAQKFLERAAVENLPTFLVELSRVLANPGNSQVARVAAGLQIKNSLTSKDPDIKAQYQQRWLAIDANARREVKNYVLQTLGTETYRPSSASQCVAGIACAEIPVNQWPELIPQLVANVTNPNSTEHMKESTLEAIGYICQDIDPEQLQ

SEQ ID NO: 13 - protein, 127 aa, synthetic construct
  REGION 1..127: note = KPNB1 polypeptide fragment
MELITILEKTVSPDRLELEAAQKFLERAAVENLPTFLVELSRVLANPGNSQVARVAAGLQIKNSLTSKDPDIKAQYQQRWLAIDANARREVKNYVLQTLGTETYRPSSASQCVAGIACAEIPVNQWP

SEQ ID NO: 14 - protein, 71 aa, synthetic construct
  REGION 1..71: note = KPNB1 polypeptide fragment
MELITILEKTVSPDRLELEAAQKFLERAAVENLPTFLVELSRVLANPGNSQVARVAAGLQIKNSLTSKDPD

SEQ ID NO: 15 - protein, 32 aa, synthetic construct
  REGION 1..32: note = KPNB1 polypeptide fragment
MELITILEKTVSPDRLELEAAQKFLERAAVEN

SEQ ID NO: 16 - protein, 480 aa, synthetic construct
  REGION 1..480: note = KPNB1 polypeptide fragment
MEPSQLKPLVIQAMPTLIELMKDPSVVVRDTAAWTVGRICELLPEAAINDVYLAPLLQCLIEGLSAEPRVASNVCWAFSSLAEAAYEAADVADDQEEPATYCLSSSFELIVQKLLETTDRPDGHQNNLRSSAYESLMEIVKNSAKDCYPAVQKTTLVIMERLQQVLQMESHIQSTSDRIQFNDLQSLLCATLQNVLRKVQHQDALQISDVVMASLLRMFQSTAGSGGVQEDALMAVSTLVEVLGGEFLKYMEAFKPFLGIGLKNYAEYQVCLAAVGLVGDLCRALQSNIIPFCDEVMQLLLENLGNENVHRSVKPQILSVFGDIALAIGGEFKKYLEVVLNTLQQASQAQVDKSDYDMVDYLNELRESCLEAYTGIVQGLKGDQENVHPDVMLVQPRVEFILSFIDHIAGDEDHTDGVVACAAGLIGDLCTAFGKDVLKLVEARPMIHELLTEGRRSKTNKAKTLATWATKELRKLKNQA

SEQ ID NO: 17 - protein, 397 aa, synthetic construct
  REGION 1..397: note = KPNB1 polypeptide fragment
MELITILERTVSPDRLELEAAQRFLERAAVENLPTFLVELSRVLANPGNSQVARVAAGLQIRNSLTSRDPDIRAQYQQRWLAIDANARREVRNYVLQTLGTETYRPSSASQCVAGIACAEIPVNQWPELIPQLVANVTNPNSTEHMRESTLEAIGYICQDIDPEQLQDRSNEILTAIIQGMRREEPSNNVRLAATNALLNSLEFTRANFDRESERHFIMQVVCEATQCPDTRVRVAALQNLVRIMSLYYQYMETYMGPALFAITIEAMRSDIDEVALQGIEFWSNVCDEEMDLAIEASEAAEQGRPPEHTSRFYARGALQYLVPILTQTLTRQDENDDDDDWNPCRAAGVCLMLLATCCEDDIVPHVLPFIREHIRNPDWRYRDAAVMAFGCILEGP

SEQ ID NO: 18 - protein, 361 aa, synthetic construct
  REGION 1..361: note = KPNB1 polypeptide fragment
MELITILERTVSPDRLELEAAQRFLERAAVENLPTFLVELSRVLANPGNSQVARVAAGLQIRNSLTSRDPDIRAQYQQRWLAIDANARREVRNYVLQTLGTETYRPSSASQCVAGIACAEIPVNQWPELIPQLVANVTNPNSTEHMRESTLEAIGYICQDIDPEQLQDRSNEILTAIIQGMRREEPSNNVRLAATNALLNSLEFTRANFDRESERHFIMQVVCEATQCPDTRVRVAALQNLVRIMSLYYQYMETYMGPALFAITIEAMRSDIDEVALQGIEFWSNVCDEEMDLAIEASEAAEQGRPPEHTSRFYARGALQYLVPILTQTLTRQDENDDDDDWNPCRAAGVCLMLLATCCED

SEQ ID NO: 19 - protein, 307 aa, synthetic construct
  REGION 1..307: note = KPNB1 polypeptide fragment
MELITILERTVSPDRLELEAAQRFLERAAVENLPTFLVELSRVLANPGNSQVARVAAGLQIRNSLTSRDPDIRAQYQQRWLAIDANARREVRNYVLQTLGTETYRPSSASQCVAGIACAEIPVNQWPELIPQLVANVTNPNSTEHMRESTLEAIGYICQDIDPEQLQDRSNEILTAIIQGMRREEPSNNVRLAATNALLNSLEFTRANFDRESERHFIMQVVCEATQCPDTRVRVAALQNLVRIMSLYYQYMETYMGPALFAITIEAMRSDIDEVALQGIEFWSNVCDEEMDLAIEASEAAEQGRPP

SEQ ID NO: 20 - protein, 249 aa, synthetic construct
  REGION 1..249: note = KPNB1 polypeptide fragment
MELITILERTVSPDRLELEAAQRFLERAAVENLPTFLVELSRVLANPGNSQVARVAAGLQIRNSLTSRDPDIRAQYQQRWLAIDANARREVRNYVLQTLGTETYRPSSASQCVAGIACAEIPVNQWPELIPQLVANVTNPNSTEHMRESTLEAIGYICQDIDPEQLQDRSNEILTAIIQGMRREEPSNNVRLAATNALLNSLEFTRANFDRESERHFIMQVVCEATQCPDTRVRVAALQNLVRIMSLYY

SEQ ID NO: 21 - protein, 209 aa, synthetic construct
  REGION 1..209: note = KPNB1 polypeptide fragment
MELITILERTVSPDRLELEAAQRFLERAAVENLPTFLVELSRVLANPGNSQVARVAAGLQIRNSLTSRDPDIRAQYQQRWLAIDANARREVRNYVLQTLGTETYRPSSASQCVAGIACAEIPVNQWPELIPQLVANVTNPNSTEHMRESTLEAIGYICQDIDPEQLQDRSNEILTAIIQGMRREEPSNNVRLAATNALLNSLEFTRANF

SEQ ID NO: 22 - protein, 167 aa, synthetic construct
  REGION 1..167: note = KPNB1 polypeptide fragment
MELITILERTVSPDRLELEAAQRFLERAAVENLPTFLVELSRVLANPGNSQVARVAAGLQIRNSLTSRDPDIRAQYQQRWLAIDANARREVRNYVLQTLGTETYRPSSASQCVAGIACAEIPVNQWPELIPQLVANVTNPNSTEHMRESTLEAIGYICQDIDPEQLQ

SEQ ID NO: 23 - protein, 127 aa, synthetic construct
  REGION 1..127: note = KPNB1 polypeptide fragment
MELITILERTVSPDRLELEAAQRFLERAAVENLPTFLVELSRVLANPGNSQVARVAAGLQIRNSLTSRDPDIRAQYQQRWLAIDANARREVRNYVLQTLGTETYRPSSASQCVAGIACAEIPVNQWP

SEQ ID NO: 24 - protein, 71 aa, synthetic construct
  REGION 1..71: note = KPNB1 polypeptide fragment
MELITILERTVSPDRLELEAAQRFLERAAVENLPTFLVELSRVLANPGNSQVARVAAGLQIRNSLTSRDPD

SEQ ID NO: 25 - protein, 32 aa, synthetic construct
  REGION 1..32: note = KPNB1 polypeptide fragment
MELITILERTVSPDRLELEAAQRFLERAAVEN

SEQ ID NO: 26 - protein, 850 aa, synthetic construct
  REGION 1..850: note = IPO3 polypeptide fragment
MNQFPDFNNYLIFVLTRLKSEDEPTRSLSGLILKNNVKAHYQSFPPPVADFIKQECLNNIGDASSLIRATIGILITTIASKGELQMWPELLPQLCNLLNSEDYNTCEGAFGALQKICEDSSELLDSDALNRPLNIMIPKFLQFFKHCSPKIRSHAIACVNQFIMDRAQALMDNIDTFIEHLFALAVDDDPEVRKNVCRALVMLLEVRIDRLIPHMHSIIQYMLQRTQDHDENVALEACEFWLTLAEQPICKEVLASHLVQLIPILVNGMKYSEIDIILLKGDVEEDEAVPDSEQDIKPRFHKSRTVTLPHEAERPDGSEDAEDDDDDDALSDWNLRKCSAAALDVLANVFREELLPHLLPLLKGLLFHPEWVVKESGILVLGAIAEGCMQGMVPYLPELIPHLIQCLSDKKALVRSIACWTLSRYAHWVVSQPPDMHLKPLMTELLKRILDGNKRVQEAACSAFATLEEEACTELVPYLSYILDTLVFAFGKYQHKNLLILYDAIGTLADSVGHHLNQPEYIQKLMPPLIQKWNELKDEDKDLFPLLECLSSVATALQSGFLPYCEPVYQRCVTLVQKTLAQAMMYTQHPEQYEAPDKDFMIVALDLLSGLAEGLGGHVEQLVARSNIMTLLFQCMQDSMPEVRQSSFALLGDLTKACFIHVKPCIAEFMPILGTNLNPEFISVCNNATWAIGEICMQMGAEMQPYVQMVLNNLVEIINRPNTPKTLLENTAITIGRLGYVCPQEVAPMLQQFIRPWCTSLRNIRDNEEKDSAFRGICMMIGVNPGGVVQDFIFFCDAVASWVSPKDDLRDMFYKILHGFKDQVGEDNWQQFSEQFPPLLKERLAAFYGV

SEQ ID NO: 27 - protein, 805 aa, synthetic construct
  REGION 1..805: note = IPO3 polypeptide fragment
MPVADFIKQECLNNIGDASSLIRATIGILITTIASKGELQMWPELLPQLCNLLNSEDYNTCEGAFGALQKICEDSSELLDSDALNRPLNIMIPKFLQFFKHCSPKIRSHAIACVNQFIMDRAQALMDNIDTFIEHLFALAVDDDPEVRKNVCRALVMLLEVRIDRLIPHMHSIIQYMLQRTQDHDENVALEACEFWLTLAEQPICKEVLASHLVQLIPILVNGMKYSEIDIILLKGDVEEDEAVPDSEQDIKPRFHKSRTVTLPHEAERPDGSEDAEDDDDDDALSDWNLRKCSAAALDVLANVFREELLPHLLPLLKGLLFHPEWVVKESGILVLGAIAEGCMQGMVPYLPELIPHLIQCLSDKKALVRSIACWTLSRYAHWVVSQPPDMHLKPLMTELLKRILDGNKRVQEAACSAFATLEEEACTELVPYLSYILDTLVFAFGKYQHKNLLILYDAIGTLADSVGHHLNQPEYIQKLMPPLIQKWNELKDEDKDLFPLLECLSSVATALQSGFLPYCEPVYQRCVTLVQKTLAQAMMYTQHPEQYEAPDKDFMIVALDLLSGLAEGLGGHVEQLVARSNIMTLLFQCMQDSMPEVRQSSFALLGDLTKACFIHVKPCIAEFMPILGTNLNPEFISVCNNATWAIGEICMQMGAEMQPYVQMVLNNLVEIINRPNTPKTLLENTAITIGRLGYVCPQEVAPMLQQFIRPWCTSLRNIRDNEEKDSAFRGICMMIGVNPGGVVQDFIFFCDAVASWVSPKDDLRDMFYKILHGFKDQVGEDNWQQFSEQFPPLLKERLAAFYGV

SEQ ID NO: 28 - protein, 765 aa, synthetic construct
  REGION 1..765: note = IPO3 polypeptide fragment
MWPELLPQLCNLLNSEDYNTCEGAFGALQKICEDSSELLDSDALNRPLNIMIPKFLQFFKHCSPKIRSHAIACVNQFIMDRAQALMDNIDTFIEHLFALAVDDDPEVRKNVCRALVMLLEVRIDRLIPHMHSIIQYMLQRTQDHDENVALEACEFWLTLAEQPICKEVLASHLVQLIPILVNGMKYSEIDIILLKGDVEEDEAVPDSEQDIKPRFHKSRTVTLPHEAERPDGSEDAEDDDDDDALSDWNLRKCSAAALDVLANVFREELLPHLLPLLKGLLFHPEWVVKESGILVLGAIAEGCMQGMVPYLPELIPHLIQCLSDKKALVRSIACWTLSRYAHWVVSQPPDMHLKPLMTELLKRILDGNKRVQEAACSAFATLEEEACTELVPYLSYILDTLVFAFGKYQHKNLLILYDAIGTLADSVGHHLNQPEYIQKLMPPLIQKWNELKDEDKDLFPLLECLSSVATALQSGFLPYCEPVYQRCVTLVQKTLAQAMMYTQHPEQYEAPDKDFMIVALDLLSGLAEGLGGHVEQLVARSNIMTLLFQCMQDSMPEVRQSSFALLGDLTKACFIHVKPCIAEFMPILGTNLNPEFISVCNNATWAIGEICMQMGAEMQPYVQMVLNNLVEIINRPNTPKTLLENTAITIGRLGYVCPQEVAPMLQQFIRPWCTSLRNIRDNEEKDSAFRGICMMIGVNPGGVVQDFIFFCDAVASWVSPKDDLRDMFYKILHGFKDQVGEDNWQQFSEQFPPLLKERLAAFYGV

SEQ ID NO: 29 - protein, 721 aa, synthetic construct
  REGION 1..721: note = IPO3 polypeptide fragment
MRPLNIMIPKFLQFFKHCSPKIRSHAIACVNQFIMDRAQALMDNIDTFIEHLFALAVDDDPEVRKNVCRALVMLLEVRIDRLIPHMHSIIQYMLQRTQDHDENVALEACEFWLTLAEQPICKEVLASHLVQLIPILVNGMKYSEIDIILLKGDVEEDEAVPDSEQDIKPRFHKSRTVTLPHEAERPDGSEDAEDDDDDDALSDWNLRKCSAAALDVLANVFREELLPHLLPLLKGLLFHPEWVVKESGILVLGAIAEGCMQGMVPYLPELIPHLIQCLSDKKALVRSIACWTLSRYAHWVVSQPPDMHLKPLMTELLKRILDGNKRVQEAACSAFATLEEEACTELVPYLSYILDTLVFAFGKYQHKNLLILYDAIGTLADSVGHHLNQPEYIQKLMPPLIQKWNELKDEDKDLFPLLECLSSVATALQSGFLPYCEPVYQRCVTLVQKTLAQAMMYTQHPEQYEAPDKDFMIVALDLLSGLAEGLGGHVEQLVARSNIMTLLFQCMQDSMPEVRQSSFALLGDLTKACFIHVKPCIAEFMPILGTNLNPEFISVCNNATWAIGEICMQMGAEMQPYVQMVLNNLVEIINRPNTPKTLLENTAITIGRLGYVCPQEVAPMLQQFIRPWCTSLRNIRDNEEKDSAFRGICMMIGVNPGGVVQDFIFFCDAVASWVSPKDDLRDMFYKILHGFKDQVGEDNWQQFSEQFPPLLKERLAAFYGV

SEQ ID NO: 30 - protein, 680 aa, synthetic construct
  REGION 1..680: note = IPO3 polypeptide fragment
MDNIDTFIEHLFALAVDDDPEVRKNVCRALVMLLEVRIDRLIPHMHSIIQYMLQRTQDHDENVALEACEFWLTLAEQPICKEVLASHLVQLIPILVNGMKYSEIDIILLKGDVEEDEAVPDSEQDIKPRFHKSRTVTLPHEAERPDGSEDAEDDDDDDALSDWNLRKCSAAALDVLANVFREELLPHLLPLLKGLLFHPEWVVKESGILVLGAIAEGCMQGMVPYLPELIPHLIQCLSDKKALVRSIACWTLSRYAHWVVSQPPDMHLKPLMTELLKRILDGNKRVQEAACSAFATLEEEACTELVPYLSYILDTLVFAFGKYQHKNLLILYDAIGTLADSVGHHLNQPEYIQKLMPPLIQKWNELKDEDKDLFPLLECLSSVATALQSGFLPYCEPVYQRCVTLVQKTLAQAMMYTQHPEQYEAPDKDFMIVALDLLSGLAEGLGGHVEQLVARSNIMTLLFQCMQDSMPEVRQSSFALLGDLTKACFIHVKPCIAEFMPILGTNLNPEFISVCNNATWAIGEICMQMGAEMQPYVQMVLNNLVEIINRPNTPKTLLENTAITIGRLGYVCPQEVAPMLQQFIRPWCTSLRNIRDNEEKDSAFRGICMMIGVNPGGVVQDFIFFCDAVASWVSPKDDLRDMFYKILHGFKDQVGEDNWQQFSEQFPPLLKERLAAFYGV

SEQ ID NO: 31 - protein, 641 aa, synthetic construct
  REGION 1..641: note = IPO3 polypeptide fragment
MLIPHMHSIIQYMLQRTQDHDENVALEACEFWLTLAEQPICKEVLASHLVQLIPILVNGMKYSEIDIILLKGDVEEDEAVPDSEQDIKPRFHKSRTVTLPHEAERPDGSEDAEDDDDDDALSDWNLRKCSAAALDVLANVFREELLPHLLPLLKGLLFHPEWVVKESGILVLGAIAEGCMQGMVPYLPELIPHLIQCLSDKKALVRSIACWTLSRYAHWVVSQPPDMHLKPLMTELLKRILDGNKRVQEAACSAFATLEEEACTELVPYLSYILDTLVFAFGKYQHKNLLILYDAIGTLADSVGHHLNQPEYIQKLMPPLIQKWNELKDEDKDLFPLLECLSSVATALQSGFLPYCEPVYQRCVTLVQKTLAQAMMYTQHPEQYEAPDKDFMIVALDLLSGLAEGLGGHVEQLVARSNIMTLLFQCMQDSMPEVRQSSFALLGDLTKACFIHVKPCIAEFMPILGTNLNPEFISVCNNATWAIGEICMQMGAEMQPYVQMVLNNLVEIINRPNTPKTLLENTAITIGRLGYVCPQEVAPMLQQFIRPWCTSLRNIRDNEEKDSAFRGICMMIGVNPGGVVQDFIFFCDAVASWVSPKDDLRDMFYKILHGFKDQVGEDNWQQFSEQFPPLLKERLAAFYGV

SEQ ID NO: 32 - protein, 602 aa, synthetic construct
  REGION 1..602: note = IPO3 polypeptide fragment
MCKEVLASHLVQLIPILVNGMKYSEIDIILLKGDVEEDEAVPDSEQDIKPRFHKSRTVTLPHEAERPDGSEDAEDDDDDDALSDWNLRKCSAAALDVLANVFREELLPHLLPLLKGLLFHPEWVVKESGILVLGAIAEGCMQGMVPYLPELIPHLIQCLSDKKALVRSIACWTLSRYAHWVVSQPPDMHLKPLMTELLKRILDGNKRVQEAACSAFATLEEEACTELVPYLSYILDTLVFAFGKYQHKNLLILYDAIGTLADSVGHHLNQPEYIQKLMPPLIQKWNELKDEDKDLFPLLECLSSVATALQSGFLPYCEPVYQRCVTLVQKTLAQAMMYTQHPEQYEAPDKDFMIVALDLLSGLAEGLGGHVEQLVARSNIMTLLFQCMQDSMPEVRQSSFALLGDLTKACFIHVKPCIAEFMPILGTNLNPEFISVCNNATWAIGEICMQMGAEMQPYVQMVLNNLVEIINRPNTPKTLLENTAITIGRLGYVCPQEVAPMLQQFIRPWCTSLRNIRDNEEKDSAFRGICMMIGVNPGGVVQDFIFFCDAVASWVSPKDDLRDMFYKILHGFKDQVGEDNWQQFSEQFPPLLKERLAAFYGV

SEQ ID NO: 33 - protein, 497 aa, synthetic construct
  REGION 1..497: note = IPO3 polypeptide fragment
MLPHLLPLLKGLLFHPEWVVKESGILVLGAIAEGCMQGMVPYLPELIPHLIQCLSDKKALVRSIACWTLSRYAHWVVSQPPDMHLKPLMTELLKRILDGNKRVQEAACSAFATLEEEACTELVPYLSYILDTLVFAFGKYQHKNLLILYDAIGTLADSVGHHLNQPEYIQKLMPPLIQKWNELKDEDKDLFPLLECLSSVATALQSGFLPYCEPVYQRCVTLVQKTLAQAMMYTQHPEQYEAPDKDFMIVALDLLSGLAEGLGGHVEQLVARSNIMTLLFQCMQDSMPEVRQSSFALLGDLTKACFIHVKPCIAEFMPILGTNLNPEFISVCNNATWAIGEICMQMGAEMQPYVQMVLNNLVEIINRPNTPKTLLENTAITIGRLGYVCPQEVAPMLQQFIRPWCTSLRNIRDNEEKDSAFRGICMMIGVNPGGVVQDFIFFCDAVASWVSPKDDLRDMFYKILHGFKDQVGEDNWQQFSEQFPPLLKERLAAFYGV

SEQ ID NO: 34 - protein, 459 aa, synthetic construct
  REGION 1..459: note = IPO3 polypeptide fragment
MVPYLPELIPHLIQCLSDKKALVRSIACWTLSRYAHWVVSQPPDMHLKPLMTELLKRILDGNKRVQEAACSAFATLEEEACTELVPYLSYILDTLVFAFGKYQHKNLLILYDAIGTLADSVGHHLNQPEYIQKLMPPLIQKWNELKDEDKDLFPLLECLSSVATALQSGFLPYCEPVYQRCVTLVQKTLAQAMMYTQHPEQYEAPDKDFMIVALDLLSGLAEGLGGHVEQLVARSNIMTLLFQCMQDSMPEVRQSSFALLGDLTKACFIHVKPCIAEFMPILGTNLNPEFISVCNNATWAIGEICMQMGAEMQPYVQMVLNNLVEIINRPNTPKTLLENTAITIGRLGYVCPQEVAPMLQQFIRPWCTSLRNIRDNEEKDSAFRGICMMIGVNPGGVVQDFIFFCDAVASWVSPKDDLRDMFYKILHGFKDQVGEDNWQQFSEQFPPLLKERLAAFYGV

SEQ ID NO: 35 - protein, 420 aa, synthetic construct
  REGION 1..420: note = IPO3 polypeptide fragment
MQPPDMHLKPLMTELLKRILDGNKRVQEAACSAFATLEEEACTELVPYLSYILDTLVFAFGKYQHKNLLILYDAIGTLADSVGHHLNQPEYIQKLMPPLIQKWNELKDEDKDLFPLLECLSSVATALQSGFLPYCEPVYQRCVTLVQKTLAQAMMYTQHPEQYEAPDKDFMIVALDLLSGLAEGLGGHVEQLVARSNIMTLLFQCMQDSMPEVRQSSFALLGDLTKACFIHVKPCIAEFMPILGTNLNPEFISVCNNATWAIGEICMQMGAEMQPYVQMVLNNLVEIINRPNTPKTLLENTAITIGRLGYVCPQEVAPMLQQFIRPWCTSLRNIRDNEEKDSAFRGICMMIGVNPGGVVQDFIFFCDAVASWVSPKDDLRDMFYKILHGFKDQVGEDNWQQFSEQFPPLLKERLAAFYGV

SEQ ID NO: 36 - protein, 376 aa, synthetic construct
  REGION 1..376: note = IPO3 polypeptide fragment
MVPYLSYILDTLVFAFGKYQHKNLLILYDAIGTLADSVGHHLNQPEYIQKLMPPLIQKWNELKDEDKDLFPLLECLSSVATALQSGFLPYCEPVYQRCVTLVQKTLAQAMMYTQHPEQYEAPDKDFMIVALDLLSGLAEGLGGHVEQLVARSNIMTLLFQCMQDSMPEVRQSSFALLGDLTKACFIHVKPCIAEFMPILGTNLNPEFISVCNNATWAIGEICMQMGAEMQPYVQMVLNNLVEIINRPNTPKTLLENTAITIGRLGYVCPQEVAPMLQQFIRPWCTSLRNIRDNEEKDSAFRGICMMIGVNPGGVVQDFIFFCDAVASWVSPKDDLRDMFYKILHGFKDQVGEDNWQQFSEQFPPLLKERLAAFYGV

SEQ ID NO: 37 - protein, 335 aa, synthetic construct
  REGION 1..335: note = IPO3 polypeptide fragment
MNQPEYIQKLMPPLIQKWNELKDEDKDLFPLLECLSSVATALQSGFLPYCEPVYQRCVTLVQKTLAQAMMYTQHPEQYEAPDKDFMIVALDLLSGLAEGLGGHVEQLVARSNIMTLLFQCMQDSMPEVRQSSFALLGDLTKACFIHVKPCIAEFMPILGTNLNPEFISVCNNATWAIGEICMQMGAEMQPYVQMVLNNLVEIINRPNTPKTLLENTAITIGRLGYVCPQEVAPMLQQFIRPWCTSLRNIRDNEEKDSAFRGICMMIGVNPGGVVQDFIFFCDAVASWVSPKDDLRDMFYKILHGFKDQVGEDNWQQFSEQFPPLLKERLAAFYGV

SEQ ID NO: 38 - protein, 289 aa, synthetic construct
  REGION 1..289: note = IPO3 polypeptide fragment
MPYCEPVYQRCVTLVQKTLAQAMMYTQHPEQYEAPDKDFMIVALDLLSGLAEGLGGHVEQLVARSNIMTLLFQCMQDSMPEVRQSSFALLGDLTKACFIHVKPCIAEFMPILGTNLNPEFISVCNNATWAIGEICMQMGAEMQPYVQMVLNNLVEIINRPNTPKTLLENTAITIGRLGYVCPQEVAPMLQQFIRPWCTSLRNIRDNEEKDSAFRGICMMIGVNPGGVVQDFIFFCDAVASWVSPKDDLRDMFYKILHGFKDQVGEDNWQQFSEQFPPLLKERLAAFYGV

SEQ ID NO: 39 - protein, 577 aa, synthetic construct
  REGION 1..577: note = IPO3 polypeptide fragment
MCKEVLASHLVQLIPILVNGMKYSEIDIILLKGDVEEDEAVPDSEQDIKPRFHKSRTVTLPHEAERPDGSEDAEDDDDDDALSDWNLRKCSAAALDVLANVFREELLPHLLPLLKGLLFHPEWVVKESGILVLGAIAEGCMQGMVPYLPELIPHLIQCLSDKKALVRSIACWTLSRYAHWVVSQPPDMHLKPLMTELLKRILDGNKRVQEAACSAFATLEEEACTELVPYLSYILDTLVFAFGKYQHKNLLILYDAIGTLADSVGHHLNQPEYIQKLMPPLIQKWNELKDEDKDLFPLLECLSSVATALQSGFLPYCEPVYQRCVTLVQKTLAQAMMYTQHPEQYEAPDKDFMIVALDLLSGLAEGLGGHVEQLVARSNIMTLLFQCMQDSMPEVRQSSFALLGDLTKACFIHVKPCIAEFMPILGTNLNPEFISVCNNATWAIGEICMQMGAEMQPYVQMVLNNLVEIINRPNTPKTLLENTAITIGRLGYVCPQEVAPMLQQFIRPWCTSLRNIRDNEEKDSAFRGICMMIGVNPGGVVQDFIFFCDAVASWVSPKDDLRDMFYKILHGFKDQVG

SEQ ID NO: 40 - protein, 537 aa, synthetic construct
  REGION 1..537: note = IPO3 polypeptide fragment
MCKEVLASHLVQLIPILVNGMKYSEIDIILLKGDVEEDEAVPDSEQDIKPRFHKSRTVTLPHEAERPDGSEDAEDDDDDDALSDWNLRKCSAAALDVLANVFREELLPHLLPLLKGLLFHPEWVVKESGILVLGAIAEGCMQGMVPYLPELIPHLIQCLSDKKALVRSIACWTLSRYAHWVVSQPPDMHLKPLMTELLKRILDGNKRVQEAACSAFATLEEEACTELVPYLSYILDTLVFAFGKYQHKNLLILYDAIGTLADSVGHHLNQPEYIQKLMPPLIQKWNELKDEDKDLFPLLECLSSVATALQSGFLPYCEPVYQRCVTLVQKTLAQAMMYTQHPEQYEAPDKDFMIVALDLLSGLAEGLGGHVEQLVARSNIMTLLFQCMQDSMPEVRQSSFALLGDLTKACFIHVKPCIAEFMPILGTNLNPEFISVCNNATWAIGEICMQMGAEMQPYVQMVLNNLVEIINRPNTPKTLLENTAITIGRLGYVCPQEVAPMLQQFIRPWCTSLRNIRDNEEKDSAFRGICMMIGVNP

SEQ ID NO: 41 - protein, 494 aa, synthetic construct
  REGION 1..494: note = IPO3 polypeptide fragment
MCKEVLASHLVQLIPILVNGMKYSEIDIILLKGDVEEDEAVPDSEQDIKPRFHKSRTVTLPHEAERPDGSEDAEDDDDDDALSDWNLRKCSAAALDVLANVFREELLPHLLPLLKGLLFHPEWVVKESGILVLGAIAEGCMQGMVPYLPELIPHLIQCLSDKKALVRSIACWTLSRYAHWVVSQPPDMHLKPLMTELLKRILDGNKRVQEAACSAFATLEEEACTELVPYLSYILDTLVFAFGKYQHKNLLILYDAIGTLADSVGHHLNQPEYIQKLMPPLIQKWNELKDEDKDLFPLLECLSSVATALQSGFLPYCEPVYQRCVTLVQKTLAQAMMYTQHPEQYEAPDKDFMIVALDLLSGLAEGLGGHVEQLVARSNIMTLLFQCMQDSMPEVRQSSFALLGDLTKACFIHVKPCIAEFMPILGTNLNPEFISVCNNATWAIGEICMQMGAEMQPYVQMVLNNLVEIINRPNTPKTLLENTAITIGRLGYVC

SEQ ID NO: 42 - protein, 457 aa, synthetic construct
  REGION 1..457: note = IPO3 polypeptide fragment
MCKEVLASHLVQLIPILVNGMKYSEIDIILLKGDVEEDEAVPDSEQDIKPRFHKSRTVTLPHEAERPDGSEDAEDDDDDDALSDWNLRKCSAAALDVLANVFREELLPHLLPLLKGLLFHPEWVVKESGILVLGAIAEGCMQGMVPYLPELIPHLIQCLSDKKALVRSIACWTLSRYAHWVVSQPPDMHLKPLMTELLKRILDGNKRVQEAACSAFATLEEEACTELVPYLSYILDTLVFAFGKYQHKNLLILYDAIGTLADSVGHHLNQPEYIQKLMPPLIQKWNELKDEDKDLFPLLECLSSVATALQSGFLPYCEPVYQRCVTLVQKTLAQAMMYTQHPEQYEAPDKDFMIVALDLLSGLAEGLGGHVEQLVARSNIMTLLFQCMQDSMPEVRQSSFALLGDLTKACFIHVKPCIAEFMPILGTNLNPEFISVCNNATWAIGEICMQMGAEMQP

SEQ ID NO: 43 - protein, 850 aa, synthetic construct
  REGION 1..850: note = IPO3 polypeptide fragment
MNQFPDFNNYLIFVLTRLRSEDEPTRSLSGLILRNNVRAHYQSFPPPVADFIRQECLNNIGDASSLIRATIGILITTIASRGELQMWPELLPQLCNLLNSEDYNTCEGAFGALQRICEDSSELLDSDALNRPLNIMIPRFLQFFRHCSPRIRSHAIACVNQFIMDRAQALMDNIDTFIEHLFALAVDDDPEVRRNVCRALVMLLEVRIDRLIPHMHSIIQYMLQRTQDHDENVALEACEFWLTLAEQPICREVLASHLVQLIPILVNGMRYSEIDIILLRGDVEEDEAVPDSEQDIRPRFHRSRTVTLPHEAERPDGSEDAEDDDDDDALSDWNLRRCSAAALDVLANVFREELLPHLLPLLRGLLFHPEWVVRESGILVLGAIAEGCMQGMVPYLPELIPHLIQCLSDRRALVRSIACWTLSRYAHWVVSQPPDMHLRPLMTELLRRILDGNRRVQEAACSAFATLEEEACTELVPYLSYILDTLVFAFGRYQHRNLLILYDAIGTLADSVGHHLNQPEYIQRLMPPLIQRWNELRDEDRDLFPLLECLSSVATALQSGFLPYCEPVYQRCVTLVQRTLAQAMMYTQHPEQYEAPDRDFMIVALDLLSGLAEGLGGHVEQLVARSNIMTLLFQCMQDSMPEVRQSSFALLGDLTRACFIHVRPCIAEFMPILGTNLNPEFISVCNNATWAIGEICMQMGAEMQPYVQMVLNNLVEIINRPNTPRTLLENTAITIGRLGYVCPQEVAPMLQQFIRPWCTSLRNIRDNEERDSAFRGICMMIGVNPGGVVQDFIFFCDAVASWVSPRDDLRDMFYRILHGFRDQVGEDNWQQFSEQFPPLLRERLAAFYGV

SEQ ID NO: 44 - protein, 805 aa, synthetic construct
  REGION 1..805: note = IPO3 polypeptide fragment
MPVADFIRQECLNNIGDASSLIRATIGILITTIASRGELQMWPELLPQLCNLLNSEDYNTCEGAFGALQRICEDSSELLDSDALNRPLNIMIPRFLQFFRHCSPRIRSHAIACVNQFIMDRAQALMDNIDTFIEHLFALAVDDDPEVRRNVCRALVMLLEVRIDRLIPHMHSIIQYMLQRTQDHDENVALEACEFWLTLAEQPICREVLASHLVQLIPILVNGMRYSEIDIILLRGDVEEDEAVPDSEQDIRPRFHRSRTVTLPHEAERPDGSEDAEDDDDDDALSDWNLRRCSAAALDVLANVFREELLPHLLPLLRGLLFHPEWVVRESGILVLGAIAEGCMQGMVPYLPELIPHLIQCLSDRRALVRSIACWTLSRYAHWVVSQPPDMHLRPLMTELLRRILDGNRRVQEAACSAFATLEEEACTELVPYLSYILDTLVFAFGRYQHRNLLILYDAIGTLADSVGHHLNQPEYIQRLMPPLIQRWNELRDEDRDLFPLLECLSSVATALQSGFLPYCEPVYQRCVTLVQRTLAQAMMYTQHPEQYEAPDRDFMIVALDLLSGLAEGLGGHVEQLVARSNIMTLLFQCMQDSMPEVRQSSFALLGDLTRACFIHVRPCIAEFMPILGTNLNPEFISVCNNATWAIGEICMQMGAEMQPYVQMVLNNLVEIINRPNTPRTLLENTAITIGRLGYVCPQEVAPMLQQFIRPWCTSLRNIRDNEERDSAFRGICMMIGVNPGGVVQDFIFFCDAVASWVSPRDDLRDMFYRILHGFRDQVGEDNWQQFSEQFPPLLRERLAAFYGV

SEQ ID NO: 45 - protein, 765 aa, synthetic construct
  REGION 1..765: note = IPO3 polypeptide fragment
MWPELLPQLCNLLNSEDYNTCEGAFGALQRICEDSSELLDSDALNRPLNIMIPRFLQFFRHCSPRIRSHAIACVNQFIMDRAQALMDNIDTFIEHLFALAVDDDPEVRRNVCRALVMLLEVRIDRLIPHMHSIIQYMLQRTQDHDENVALEACEFWLTLAEQPICREVLASHLVQLIPILVNGMRYSEIDIILLRGDVEEDEAVPDSEQDIRPRFHRSRTVTLPHEAERPDGSEDAEDDDDDDALSDWNLRRCSAAALDVLANVFREELLPHLLPLLRGLLFHPEWVVRESGILVLGAIAEGCMQGMVPYLPELIPHLIQCLSDRRALVRSIACWTLSRYAHWVVSQPPDMHLRPLMTELLRRILDGNRRVQEAACSAFATLEEEACTELVPYLSYILDTLVFAFGRYQHRNLLILYDAIGTLADSVGHHLNQPEYIQRLMPPLIQRWNELRDEDRDLFPLLECLSSVATALQSGFLPYCEPVYQRCVTLVQRTLAQAMMYTQHPEQYEAPDRDFMIVALDLLSGLAEGLGGHVEQLVARSNIMTLLFQCMQDSMPEVRQSSFALLGDLTRACFIHVRPCIAEFMPILGTNLNPEFISVCNNATWAIGEICMQMGAEMQPYVQMVLNNLVEIINRPNTPRTLLENTAITIGRLGYVCPQEVAPMLQQFIRPWCTSLRNIRDNEERDSAFRGICMMIGVNPGGVVQDFIFFCDAVASWVSPRDDLRDMFYRILHGFRDQVGEDNWQQFSEQFPPLLRERLAAFYGV

SEQ ID NO: 46 - protein, 721 aa, synthetic construct
  REGION 1..721: note = IPO3 polypeptide fragment
MRPLNIMIPRFLQFFRHCSPRIRSHAIACVNQFIMDRAQALMDNIDTFIEHLFALAVDDDPEVRRNVCRALVMLLEVRIDRLIPHMHSIIQYMLQRTQDHDENVALEACEFWLTLAEQPICREVLASHLVQLIPILVNGMRYSEIDIILLRGDVEEDEAVPDSEQDIRPRFHRSRTVTLPHEAERPDGSEDAEDDDDDDALSDWNLRRCSAAALDVLANVFREELLPHLLPLLRGLLFHPEWVVRESGILVLGAIAEGCMQGMVPYLPELIPHLIQCLSDRRALVRSIACWTLSRYAHWVVSQPPDMHLRPLMTELLRRILDGNRRVQEAACSAFATLEEEACTELVPYLSYILDTLVFAFGRYQHRNLLILYDAIGTLADSVGHHLNQPEYIQRLMPPLIQRWNELRDEDRDLFPLLECLSSVATALQSGFLPYCEPVYQRCVTLVQRTLAQAMMYTQHPEQYEAPDRDFMIVALDLLSGLAEGLGGHVEQLVARSNIMTLLFQCMQDSMPEVRQSSFALLGDLTRACFIHVRPCIAEFMPILGTNLNPEFISVCNNATWAIGEICMQMGAEMQPYVQMVLNNLVEIINRPNTPRTLLENTAITIGRLGYVCPQEVAPMLQQFIRPWCTSLRNIRDNEERDSAFRGICMMIGVNPGGVVQDFIFFCDAVASWVSPRDDLRDMFYRILHGFRDQVGEDNWQQFSEQFPPLLRERLAAFYGV

SEQ ID NO: 47 - protein, 680 aa, synthetic construct
  REGION 1..680: note = IPO3 polypeptide fragment
MDNIDTFIEHLFALAVDDDPEVRRNVCRALVMLLEVRIDRLIPHMHSIIQYMLQRTQDHDENVALEACEFWLTLAEQPICREVLASHLVQLIPILVNGMRYSEIDIILLRGDVEEDEAVPDSEQDIRPRFHRSRTVTLPHEAERPDGSEDAEDDDDDDALSDWNLRRCSAAALDVLANVFREELLPHLLPLLRGLLFHPEWVVRESGILVLGAIAEGCMQGMVPYLPELIPHLIQCLSDRRALVRSIACWTLSRYAHWVVSQPPDMHLRPLMTELLRRILDGNRRVQEAACSAFATLEEEACTELVPYLSYILDTLVFAFGRYQHRNLLILYDAIGTLADSVGHHLNQPEYIQRLMPPLIQRWNELRDEDRDLFPLLECLSSVATALQSGFLPYCEPVYQRCVTLVQRTLAQAMMYTQHPEQYEAPDRDFMIVALDLLSGLAEGLGGHVEQLVARSNIMTLLFQCMQDSMPEVRQSSFALLGDLTRACFIHVRPCIAEFMPILGTNLNPEFISVCNNATWAIGEICMQMGAEMQPYVQMVLNNLVEIINRPNTPRTLLENTAITIGRLGYVCPQEVAPMLQQFIRPWCTSLRNIRDNEERDSAFRGICMMIGVNPGGVVQDFIFFCDAVASWVSPRDDLRDMFYRILHGFRDQVGEDNWQQFSEQFPPLLRERLAAFYGV

SEQ ID NO: 48 - protein, 641 aa, synthetic construct
  REGION 1..641: note = IPO3 polypeptide fragment
MLIPHMHSIIQYMLQRTQDHDENVALEACEFWLTLAEQPICREVLASHLVQLIPILVNGMRYSEIDIILLRGDVEEDEAVPDSEQDIRPRFHRSRTVTLPHEAERPDGSEDAEDDDDDDALSDWNLRRCSAAALDVLANVFREELLPHLLPLLRGLLFHPEWVVRESGILVLGAIAEGCMQGMVPYLPELIPHLIQCLSDRRALVRSIACWTLSRYAHWVVSQPPDMHLRPLMTELLRRILDGNRRVQEAACSAFATLEEEACTELVPYLSYILDTLVFAFGRYQHRNLLILYDAIGTLADSVGHHLNQPEYIQRLMPPLIQRWNELRDEDRDLFPLLECLSSVATALQSGFLPYCEPVYQRCVTLVQRTLAQAMMYTQHPEQYEAPDRDFMIVALDLLSGLAEGLGGHVEQLVARSNIMTLLFQCMQDSMPEVRQSSFALLGDLTRACFIHVRPCIAEFMPILGTNLNPEFISVCNNATWAIGEICMQMGAEMQPYVQMVLNNLVEIINRPNTPRTLLENTAITIGRLGYVCPQEVAPMLQQFIRPWCTSLRNIRDNEERDSAFRGICMMIGVNPGGVVQDFIFFCDAVASWVSPRDDLRDMFYRILHGFRDQVGEDNWQQFSEQFPPLLRERLAAFYGV

SEQ ID NO: 49 - protein, 602 aa, synthetic construct
  REGION 1..602: note = IPO3 polypeptide fragment
MCREVLASHLVQLIPILVNGMRYSEIDIILLRGDVEEDEAVPDSEQDIRPRFHRSRTVTLPHEAERPDGSEDAEDDDDDDALSDWNLRRCSAAALDVLANVFREELLPHLLPLLRGLLFHPEWVVRESGILVLGAIAEGCMQGMVPYLPELIPHLIQCLSDRRALVRSIACWTLSRYAHWVVSQPPDMHLRPLMTELLRRILDGNRRVQEAACSAFATLEEEACTELVPYLSYILDTLVFAFGRYQHRNLLILYDAIGTLADSVGHHLNQPEYIQRLMPPLIQRWNELRDEDRDLFPLLECLSSVATALQSGFLPYCEPVYQRCVTLVQRTLAQAMMYTQHPEQYEAPDRDFMIVALDLLSGLAEGLGGHVEQLVARSNIMTLLFQCMQDSMPEVRQSSFALLGDLTRACFIHVRPCIAEFMPILGTNLNPEFISVCNNATWAIGEICMQMGAEMQPYVQMVLNNLVEIINRPNTPRTLLENTAITIGRLGYVCPQEVAPMLQQFIRPWCTSLRNIRDNEERDSAFRGICMMIGVNPGGVVQDFIFFCDAVASWVSPRDDLRDMFYRILHGFRDQVGEDNWQQFSEQFPPLLRERLAAFYGV

SEQ ID NO: 50 - protein, 497 aa, synthetic construct
  REGION 1..497: note = IPO3 polypeptide fragment
MLPHLLPLLRGLLFHPEWVVRESGILVLGAIAEGCMQGMVPYLPELIPHLIQCLSDRRALVRSIACWTLSRYAHWVVSQPPDMHLRPLMTELLRRILDGNRRVQEAACSAFATLEEEACTELVPYLSYILDTLVFAFGRYQHRNLLILYDAIGTLADSVGHHLNQPEYIQRLMPPLIQRWNELRDEDRDLFPLLECLSSVATALQSGFLPYCEPVYQRCVTLVQRTLAQAMMYTQHPEQYEAPDRDFMIVALDLLSGLAEGLGGHVEQLVARSNIMTLLFQCMQDSMPEVRQSSFALLGDLTRACFIHVRPCIAEFMPILGTNLNPEFISVCNNATWAIGEICMQMGAEMQPYVQMVLNNLVEIINRPNTPRTLLENTAITIGRLGYVCPQEVAPMLQQFIRPWCTSLRNIRDNEERDSAFRGICMMIGVNPGGVVQDFIFFCDAVASWVSPRDDLRDMFYRILHGFRDQVGEDNWQQFSEQFPPLLRERLAAFYGV

SEQ ID NO: 51 - protein, 459 aa, synthetic construct
  REGION 1..459: note = IPO3 polypeptide fragment
MVPYLPELIPHLIQCLSDRRALVRSIACWTLSRYAHWVVSQPPDMHLRPLMTELLRRILDGNRRVQEAACSAFATLEEEACTELVPYLSYILDTLVFAFGRYQHRNLLILYDAIGTLADSVGHHLNQPEYIQRLMPPLIQRWNELRDEDRDLFPLLECLSSVATALQSGFLPYCEPVYQRCVTLVQRTLAQAMMYTQHPEQYEAPDRDFMIVALDLLSGLAEGLGGHVEQLVARSNIMTLLFQCMQDSMPEVRQSSFALLGDLTRACFIHVRPCIAEFMPILGTNLNPEFISVCNNATWAIGEICMQMGAEMQPYVQMVLNNLVEIINRPNTPRTLLENTAITIGRLGYVCPQEVAPMLQQFIRPWCTSLRNIRDNEERDSAFRGICMMIGVNPGGVVQDFIFFCDAVASWVSPRDDLRDMFYRILHGFRDQVGEDNWQQFSEQFPPLLRERLAAFYGV

SEQ ID NO: 52 - protein, 420 aa, synthetic construct
  REGION 1..420: note = IPO3 polypeptide fragment
MQPPDMHLRPLMTELLRRILDGNRRVQEAACSAFATLEEEACTELVPYLSYILDTLVFAFGRYQHRNLLILYDAIGTLADSVGHHLNQPEYIQRLMPPLIQRWNELRDEDRDLFPLLECLSSVATALQSGFLPYCEPVYQRCVTLVQRTLAQAMMYTQHPEQYEAPDRDFMIVALDLLSGLAEGLGGHVEQLVARSNIMTLLFQCMQDSMPEVRQSSFALLGDLTRACFIHVRPCIAEFMPILGTNLNPEFISVCNNATWAIGEICMQMGAEMQPYVQMVLNNLVEIINRPNTPRTLLENTAITIGRLGYVCPQEVAPMLQQFIRPWCTSLRNIRDNEERDSAFRGICMMIGVNPGGVVQDFIFFCDAVASWVSPRDDLRDMFYRILHGFRDQVGEDNWQQFSEQFPPLLRERLAAFYGV

SEQ ID NO: 53 - protein, 376 aa, synthetic construct
  REGION 1..376: note = IPO3 polypeptide fragment
MVPYLSYILDTLVFAFGRYQHRNLLILYDAIGTLADSVGHHLNQPEYIQRLMPPLIQRWNELRDEDRDLFPLLECLSSVATALQSGFLPYCEPVYQRCVTLVQRTLAQAMMYTQHPEQYEAPDRDFMIVALDLLSGLAEGLGGHVEQLVARSNIMTLLFQCMQDSMPEVRQSSFALLGDLTRACFIHVRPCIAEFMPILGTNLNPEFISVCNNATWAIGEICMQMGAEMQPYVQMVLNNLVEIINRPNTPRTLLENTAITIGRLGYVCPQEVAPMLQQFIRPWCTSLRNIRDNEERDSAFRGICMMIGVNPGGVVQDFIFFCDAVASWVSPRDDLRDMFYRILHGFRDQVGEDNWQQFSEQFPPLLRERLAAFYGV

SEQ ID NO: 54 - protein, 335 aa, synthetic construct
  REGION 1..335: note = IPO3 polypeptide fragment
MNQPEYIQRLMPPLIQRWNELRDEDRDLFPLLECLSSVATALQSGFLPYCEPVYQRCVTLVQRTLAQAMMYTQHPEQYEAPDRDFMIVALDLLSGLAEGLGGHVEQLVARSNIMTLLFQCMQDSMPEVRQSSFALLGDLTRACFIHVRPCIAEFMPILGTNLNPEFISVCNNATWAIGEICMQMGAEMQPYVQMVLNNLVEIINRPNTPRTLLENTAITIGRLGYVCPQEVAPMLQQFIRPWCTSLRNIRDNEERDSAFRGICMMIGVNPGGVVQDFIFFCDAVASWVSPRDDLRDMFYRILHGFRDQVGEDNWQQFSEQFPPLLRERLAAFYGV

SEQ ID NO: 55 - protein, 289 aa, synthetic construct
  REGION 1..289: note = IPO3 polypeptide fragment
MPYCEPVYQRCVTLVQRTLAQAMMYTQHPEQYEAPDRDFMIVALDLLSGLAEGLGGHVEQLVARSNIMTLLFQCMQDSMPEVRQSSFALLGDLTRACFIHVRPCIAEFMPILGTNLNPEFISVCNNATWAIGEICMQMGAEMQPYVQMVLNNLVEIINRPNTPRTLLENTAITIGRLGYVCPQEVAPMLQQFIRPWCTSLRNIRDNEERDSAFRGICMMIGVNPGGVVQDFIFFCDAVASWVSPRDDLRDMFYRILHGFRDQVGEDNWQQFSEQFPPLLRERLAAFYGV

SEQ ID NO: 56 - protein, 942 aa, synthetic construct
  REGION 1..942: note = IPO13 polypeptide fragment
MVENVEKALHQLYYDPNIENKNLAQKWLMQAQVSPQAWHFSWQLLQPDKVPEIQYFGASALHIKISRYWSDIPTDQYESLKAQLFTQITRFASGSKIVLTRLCVALASLALSMMPDAWPCAVADMVRLFQAEDSPVDGQGRCLALLELLTVLPEEFQTSRLPQYRKGLVRTSLAVECGAVFPLLEQLLQQPSSPSCVRQKVLKCFSSWVQLEVPLQDCEALIQAAFAALQDSELFDSSVEAIVNAISQPDAQRYVNTLLKLIPLVLGLQEQLRQAVQNGDMETSHGICRIAVALGENHSRALLDQVEHWQSFLALVNMIMFCTGIPGHYPVNETTSSLTLTFWYTLQDDILSFEAEKQAVYQQVYRPVYFQLVDVLLHKAQFPSDEEYGFWSSDEKEQFRIYRVDISDTLMYVYEMLGAELLSNLYDKLGRLLTSSEEPYSWQHTEALLYGFQSIAETIDVNYSDVVPGLIGLIPRISISNVQLADTVMFTIGALSEWLADHPVMINSVLPLVLHALGNPELSVSSVSTLKKICRECKYDLPPYAANIVAVSQDVLMKQIHKTSQCMWLMQALGFLLSALQVEEILKNLHSLISPYIQQLEKLAEEIPNPSNKLAIVHILGLLSNLFTTLDISHHEDDHEGPELRKLPVPQGPNPVVVVLQQVFQLIQKVLSKWLNDAQVVEAVCAIFEKSVKTLLDDFAPMVPQLCEMLGRMYSTIPQASALDLTRQLVHIFAHEPAHFPPIEALFLLVTSVTLTLFQQGPRDHPDIVDSFMQLLAQALKRKPDLFLCERLDVKSVFQCAVLALKFPEAPTVKASCGFFTELLPRCGEVESVGKVVQEDGRMLLIAVLEAIGGQASRSLMDCFADILFALNKHCFSLLSMWIKEALQPPGFPSARLSPEQKDTFSQQILRERVNKRRVKEMVKEFTLLCRGLHGTDYTADY

SEQ ID NO: 57 - protein, 908 aa, synthetic construct
  REGION 1..908: note = IPO13 polypeptide fragment
MQAWHFSWQLLQPDKVPEIQYFGASALHIKISRYWSDIPTDQYESLKAQLFTQITRFASGSKIVLTRLCVALASLALSMMPDAWPCAVADMVRLFQAEDSPVDGQGRCLALLELLTVLPEEFQTSRLPQYRKGLVRTSLAVECGAVFPLLEQLLQQPSSPSCVRQKVLKCFSSWVQLEVPLQDCEALIQAAFAALQDSELFDSSVEAIVNAISQPDAQRYVNTLLKLIPLVLGLQEQLRQAVQNGDMETSHGICRIAVALGENHSRALLDQVEHWQSFLALVNMIMFCTGIPGHYPVNETTSSLTLTFWYTLQDDILSFEAEKQAVYQQVYRPVYFQLVDVLLHKAQFPSDEEYGFWSSDEKEQFRIYRVDISDTLMYVYEMLGAELLSNLYDKLGRLLTSSEEPYSWQHTEALLYGFQSIAETIDVNYSDVVPGLIGLIPRISISNVQLADTVMFTIGALSEWLADHPVMINSVLPLVLHALGNPELSVSSVSTLKKICRECKYDLPPYAANIVAVSQDVLMKQIHKTSQCMWLMQALGFLLSALQVEEILKNLHSLISPYIQQLEKLAEEIPNPSNKLAIVHILGLLSNLFTTLDISHHEDDHEGPELRKLPVPQGPNPVVVVLQQVFQLIQKVLSKWLNDAQVVEAVCAIFEKSVKTLLDDFAPMVPQLCEMLGRMYSTIPQASALDLTRQLVHIFAHEPAHFPPIEALFLLVTSVTLTLFQQGPRDHPDIVDSFMQLLAQALKRKPDLFLCERLDVKSVFQCAVLALKFPEAPTVKASCGFFTELLPRCGEVESVGKVVQEDGRMLLIAVLEAIGGQASRSLMDCFADILFALNKHCFSLLSMWIKEALQPPGFPSARLSPEQKDTFSQQILRERVNKRRVKEMVKEFTLLCRGLHGTDYTADY

SEQ ID NO: 58 - protein, 872 aa, synthetic construct
  REGION 1..872: note = IPO13 polypeptide fragment
MIPTDQYESLKAQLFTQITRFASGSKIVLTRLCVALASLALSMMPDAWPCAVADMVRLFQAEDSPVDGQGRCLALLELLTVLPEEFQTSRLPQYRKGLVRTSLAVECGAVFPLLEQLLQQPSSPSCVRQKVLKCFSSWVQLEVPLQDCEALIQAAFAALQDSELFDSSVEAIVNAISQPDAQRYVNTLLKLIPLVLGLQEQLRQAVQNGDMETSHGICRIAVALGENHSRALLDQVEHWQSFLALVNMIMFCTGIPGHYPVNETTSSLTLTFWYTLQDDILSFEAEKQAVYQQVYRPVYFQLVDVLLHKAQFPSDEEYGFWSSDEKEQFRIYRVDISDTLMYVYEMLGAELLSNLYDKLGRLLTSSEEPYSWQHTEALLYGFQSIAETIDVNYSDVVPGLIGLIPRISISNVQLADTVMFTIGALSEWLADHPVMINSVLPLVLHALGNPELSVSSVSTLKKICRECKYDLPPYAANIVAVSQDVLMKQIHKTSQCMWLMQALGFLLSALQVEEILKNLHSLISPYIQQLEKLAEEIPNPSNKLAIVHILGLLSNLFTTLDISHHEDDHEGPELRKLPVPQGPNPVVVVLQQVFQLIQKVLSKWLNDAQVVEAVCAIFEKSVKTLLDDFAPMVPQLCEMLGRMYSTIPQASALDLTRQLVHIFAHEPAHFPPIEALFLLVTSVTLTLFQQGPRDHPDIVDSFMQLLAQALKRKPDLFLCERLDVKSVFQCAVLALKFPEAPTVKASCGFFTELLPRCGEVESVGKVVQEDGRMLLIAVLEAIGGQASRSLMDCFADILFALNKHCFSLLSMWIKEALQPPGFPSARLSPEQKDTFSQQILRERVNKRRVKEMVKEFTLLCRGLHGTDYTADY

SEQ ID NO: 59 - protein, 826 aa, synthetic construct
  REGION 1..826: note = IPO13 polypeptide fragment
MWPCAVADMVRLFQAEDSPVDGQGRCLALLELLTVLPEEFQTSRLPQYRKGLVRTSLAVECGAVFPLLEQLLQQPSSPSCVRQKVLKCFSSWVQLEVPLQDCEALIQAAFAALQDSELFDSSVEAIVNAISQPDAQRYVNTLLKLIPLVLGLQEQLRQAVQNGDMETSHGICRIAVALGENHSRALLDQVEHWQSFLALVNMIMFCTGIPGHYPVNETTSSLTLTFWYTLQDDILSFEAEKQAVYQQVYRPVYFQLVDVLLHKAQFPSDEEYGFWSSDEKEQFRIYRVDISDTLMYVYEMLGAELLSNLYDKLGRLLTSSEEPYSWQHTEALLYGFQSIAETIDVNYSDVVPGLIGLIPRISISNVQLADTVMFTIGALSEWLADHPVMINSVLPLVLHALGNPELSVSSVSTLKKICRECKYDLPPYAANIVAVSQDVLMKQIHKTSQCMWLMQALGFLLSALQVEEILKNLHSLISPYIQQLEKLAEEIPNPSNKLAIVHILGLLSNLFTTLDISHHEDDHEGPELRKLPVPQGPNPVVVVLQQVFQLIQKVLSKWLNDAQVVEAVCAIFEKSVKTLLDDFAPMVPQLCEMLGRMYSTIPQASALDLTRQLVHIFAHEPAHFPPIEALFLLVTSVTLTLFQQGPRDHPDIVDSFMQLLAQALKRKPDLFLCERLDVKSVFQCAVLALKFPEAPTVKASCGFFTELLPRCGEVESVGKVVQEDGRMLLIAVLEAIGGQASRSLMDCFADILFALNKHCFSLLSMWIKEALQPPGFPSARLSPEQKDTFSQQILRERVNKRRVKEMVKEFTLLCRGLHGTDYTADY

SEQ ID NO: 60 - protein, 783 aa, synthetic construct
  REGION 1..783: note = IPO13 polypeptide fragment
MLPQYRKGLVRTSLAVECGAVFPLLEQLLQQPSSPSCVRQKVLKCFSSWVQLEVPLQDCEALIQAAFAALQDSELFDSSVEAIVNAISQPDAQRYVNTLLKLIPLVLGLQEQLRQAVQNGDMETSHGICRIAVALGENHSRALLDQVEHWQSFLALVNMIMFCTGIPGHYPVNETTSSLTLTFWYTLQDDILSFEAEKQAVYQQVYRPVYFQLVDVLLHKAQFPSDEEYGFWSSDEKEQFRIYRVDISDTLMYVYEMLGAELLSNLYDKLGRLLTSSEEPYSWQHTEALLYGFQSIAETIDVNYSDVVPGLIGLIPRISISNVQLADTVMFTIGALSEWLADHPVMINSVLPLVLHALGNPELSVSSVSTLKKICRECKYDLPPYAANIVAVSQDVLMKQIHKTSQCMWLMQALGFLLSALQVEEILKNLHSLISPYIQQLEKLAEEIPNPSNKLAIVHILGLLSNLFTTLDISHHEDDHEGPELRKLPVPQGPNPVVVVLQQVFQLIQKVLSKWLNDAQVVEAVCAIFEKSVKTLLDDFAPMVPQLCEMLGRMYSTIPQASALDLTRQLVHIFAHEPAHFPPIEALFLLVTSVTLTLFQQGPRDHPDIVDSFMQLLAQALKRKPDLFLCERLDVKSVFQCAVLALKFPEAPTVKASCGFFTELLPRCGEVESVGKVVQEDGRMLLIAVLEAIGGQASRSLMDCFADILFALNKHCFSLLSMWIKEALQPPGFPSARLSPEQKDTFSQQILRERVNKRRVKEMVKEFTLLCRGLHGTDYTADY

SEQ ID NO: 61 - protein, 732 aa, synthetic construct
  REGION 1..732: note = IPO13 polypeptide fragment
MEVPLQDCEALIQAAFAALQDSELFDSSVEAIVNAISQPDAQRYVNTLLKLIPLVLGLQEQLRQAVQNGDMETSHGICRIAVALGENHSRALLDQVEHWQSFLALVNMIMFCTGIPGHYPVNETTSSLTLTFWYTLQDDILSFEAEKQAVYQQVYRPVYFQLVDVLLHKAQFPSDEEYGFWSSDEKEQFRIYRVDISDTLMYVYEMLGAELLSNLYDKLGRLLTSSEEPYSWQHTEALLYGFQSIAETIDVNYSDVVPGLIGLIPRISISNVQLADTVMFTIGALSEWLADHPVMINSVLPLVLHALGNPELSVSSVSTLKKICRECKYDLPPYAANIVAVSQDVLMKQIHKTSQCMWLMQALGFLLSALQVEEILKNLHSLISPYIQQLEKLAEEIPNPSNKLAIVHILGLLSNLFTTLDISHHEDDHEGPELRKLPVPQGPNPVVVVLQQVFQLIQKVLSKWLNDAQVVEAVCAIFEKSVKTLLDDFAPMVPQLCEMLGRMYSTIPQASALDLTRQLVHIFAHEPAHFPPIEALFLLVTSVTLTLFQQGPRDHPDIVDSFMQLLAQALKRKPDLFLCERLDVKSVFQCAVLALKFPEAPTVKASCGFFTELLPRCGEVESVGKVVQEDGRMLLIAVLEAIGGQASRSLMDCFADILFALNKHCFSLLSMWIKEALQPPGFPSARLSPEQKDTFSQQILRERVNKRRVKEMVKEFTLLCRGLHGTDYTADY

SEQ ID NO: 62 - protein, 488 aa, synthetic construct
  REGION 1..488: note = IPO13 polypeptide fragment
MAETIDVNYSDVVPGLIGLIPRISISNVQLADTVMFTIGALSEWLADHPVMINSVLPLVLHALGNPELSVSSVSTLKKICRECKYDLPPYAANIVAVSQDVLMKQIHKTSQCMWLMQALGFLLSALQVEEILKNLHSLISPYIQQLEKLAEEIPNPSNKLAIVHILGLLSNLFTTLDISHHEDDHEGPELRKLPVPQGPNPVVVVLQQVFQLIQKVLSKWLNDAQVVEAVCAIFEKSVKTLLDDFAPMVPQLCEMLGRMYSTIPQASALDLTRQLVHIFAHEPAHFPPIEALFLLVTSVTLTLFQQGPRDHPDIVDSFMQLLAQALKRKPDLFLCERLDVKSVFQCAVLALKFPEAPTVKASCGFFTELLPRCGEVESVGKVVQEDGRMLLIAVLEAIGGQASRSLMDCFADILFALNKHCFSLLSMWIKEALQPPGFPSARLSPEQKDTFSQQILRERVNKRRVKEMVKEFTLLCRGLHGTDYTADY

SEQ ID NO: 63 - protein, 933 aa, synthetic construct
  REGION 1..933: note = IPO13 polypeptide fragment
MERREEQPGAAGAGAAPALDFTVENVEKALHQLYYDPNIENKNLAQKWLMQAQVSPQAWHFSWQLLQPDKVPEIQYFGASALHIKISRYWSDIPTDQYESLKAQLFTQITRFASGSKIVLTRLCVALASLALSMMPDAWPCAVADMVRLFQAEDSPVDGQGRCLALLELLTVLPEEFQTSRLPQYRKGLVRTSLAVECGAVFPLLEQLLQQPSSPSCVRQKVLKCFSSWVQLEVPLQDCEALIQAAFAALQDSELFDSSVEAIVNAISQPDAQRYVNTLLKLIPLVLGLQEQLRQAVQNGDMETSHGICRIAVALGENHSRALLDQVEHWQSFLALVNMIMFCTGIPGHYPVNETTSSLTLTFWYTLQDDILSFEAEKQAVYQQVYRPVYFQLVDVLLHKAQFPSDEEYGFWSSDEKEQFRIYRVDISDTLMYVYEMLGAELLSNLYDKLGRLLTSSEEPYSWQHTEALLYGFQSIAETIDVNYSDVVPGLIGLIPRISISNVQLADTVMFTIGALSEWLADHPVMINSVLPLVLHALGNPELSVSSVSTLKKICRECKYDLPPYAANIVAVSQDVLMKQIHKTSQCMWLMQALGFLLSALQVEEILKNLHSLISPYIQQLEKLAEEIPNPSNKLAIVHILGLLSNLFTTLDISHHEDDHEGPELRKLPVPQGPNPVVVVLQQVFQLIQKVLSKWLNDAQVVEAVCAIFEKSVKTLLDDFAPMVPQLCEMLGRMYSTIPQASALDLTRQLVHIFAHEPAHFPPIEALFLLVTSVTLTLFQQGPRDHPDIVDSFMQLLAQALKRKPDLFLCERLDVKSVFQCAVLALKFPEAPTVKASCGFFTELLPRCGEVESVGKVVQEDGRMLLIAVLEAIGGQASRSLMDCFADILFALNKHCFSLLSMWIKEALQPPGFPSARLSPEQKDTFSQQILRE

SEQ ID NO: 64 - protein, 896 aa, synthetic construct
  REGION 1..896: note = IPO13 polypeptide fragment
MERREEQPGAAGAGAAPALDFTVENVEKALHQLYYDPNIENKNLAQKWLMQAQVSPQAWHFSWQLLQPDKVPEIQYFGASALHIKISRYWSDIPTDQYESLKAQLFTQITRFASGSKIVLTRLCVALASLALSMMPDAWPCAVADMVRLFQAEDSPVDGQGRCLALLELLTVLPEEFQTSRLPQYRKGLVRTSLAVECGAVFPLLEQLLQQPSSPSCVRQKVLKCFSSWVQLEVPLQDCEALIQAAFAALQDSELFDSSVEAIVNAISQPDAQRYVNTLLKLIPLVLGLQEQLRQAVQNGDMETSHGICRIAVALGENHSRALLDQVEHWQSFLALVNMIMFCTGIPGHYPVNETTSSLTLTFWYTLQDDILSFEAEKQAVYQQVYRPVYFQLVDVLLHKAQFPSDEEYGFWSSDEKEQFRIYRVDISDTLMYVYEMLGAELLSNLYDKLGRLLTSSEEPYSWQHTEALLYGFQSIAETIDVNYSDVVPGLIGLIPRISISNVQLADTVMFTIGALSEWLADHPVMINSVLPLVLHALGNPELSVSSVSTLKKICRECKYDLPPYAANIVAVSQDVLMKQIHKTSQCMWLMQALGFLLSALQVEEILKNLHSLISPYIQQLEKLAEEIPNPSNKLAIVHILGLLSNLFTTLDISHHEDDHEGPELRKLPVPQGPNPVVVVLQQVFQLIQKVLSKWLNDAQVVEAVCAIFEKSVKTLLDDFAPMVPQLCEMLGRMYSTIPQASALDLTRQLVHIFAHEPAHFPPIEALFLLVTSVTLTLFQQGPRDHPDIVDSFMQLLAQALKRKPDLFLCERLDVKSVFQCAVLALKFPEAPTVKASCGFFTELLPRCGEVESVGKVVQEDGRMLLIAVLEAIGGQASRSLMDCFADILFALNKHC

SEQ ID NO: 65 - protein, 476 aa, synthetic construct
  REGION 1..476: note = IPO13 polypeptide fragment
MERREEQPGAAGAGAAPALDFTVENVEKALHQLYYDPNIENKNLAQKWLMQAQVSPQAWHFSWQLLQPDKVPEIQYFGASALHIKISRYWSDIPTDQYESLKAQLFTQITRFASGSKIVLTRLCVALASLALSMMPDAWPCAVADMVRLFQAEDSPVDGQGRCLALLELLTVLPEEFQTSRLPQYRKGLVRTSLAVECGAVFPLLEQLLQQPSSPSCVRQKVLKCFSSWVQLEVPLQDCEALIQAAFAALQDSELFDSSVEAIVNAISQPDAQRYVNTLLKLIPLVLGLQEQLRQAVQNGDMETSHGICRIAVALGENHSRALLDQVEHWQSFLALVNMIMFCTGIPGHYPVNETTSSLTLTFWYTLQDDILSFEAEKQAVYQQVYRPVYFQLVDVLLHKAQFPSDEEYGFWSSDEKEQFRIYRVDISDTLMYVYEMLGAELLSNLYDKLGRLLTSSEEPYSWQHTEALLYGFQSI

SEQ ID NO: 66 - protein, 523 aa, synthetic construct
  REGION 1..523: note = IPO13 polypeptide fragment
MERREEQPGAAGAGAAPALDFTVENVEKALHQLYYDPNIENKNLAQKWLMQAQVSPQAWHFSWQLLQPDKVPEIQYFGASALHIKISRYWSDIPTDQYESLKAQLFTQITRFASGSKIVLTRLCVALASLALSMMPDAWPCAVADMVRLFQAEDSPVDGQGRCLALLELLTVLPEEFQTSRLPQYRKGLVRTSLAVECGAVFPLLEQLLQQPSSPSCVRQKVLKCFSSWVQLEVPLQDCEALIQAAFAALQDSELFDSSVEAIVNAISQPDAQRYVNTLLKLIPLVLGLQEQLRQAVQNGDMETSHGICRIAVALGENHSRALLDQVEHWQSFLALVNMIMFCTGIPGHYPVNETTSSLTLTFWYTLQDDILSFEAEKQAVYQQVYRPVYFQLVDVLLHKAQFPSDEEYGFWSSDEKEQFRIYRVDISDTLMYVYEMLGAELLSNLYDKLGRLLTSSEEPYSWQHTEALLYGFQSIAETIDVNYSDVVPGLIGLIPRISISNVQLADTVMFTIGALSEWLADH

SEQ ID NO: 67 - protein, 942 aa, synthetic construct
  REGION 1..942: note = IPO13 polypeptide fragment
MVENVERALHQLYYDPNIENRNLAQRWLMQAQVSPQAWHFSWQLLQPDRVPEIQYFGASALHIRISRYWSDIPTDQYESLRAQLFTQITRFASGSRIVLTRLCVALASLALSMMPDAWPCAVADMVRLFQAEDSPVDGQGRCLALLELLTVLPEEFQTSRLPQYRRGLVRTSLAVECGAVFPLLEQLLQQPSSPSCVRQRVLRCFSSWVQLEVPLQDCEALIQAAFAALQDSELFDSSVEAIVNAISQPDAQRYVNTLLRLIPLVLGLQEQLRQAVQNGDMETSHGICRIAVALGENHSRALLDQVEHWQSFLALVNMIMFCTGIPGHYPVNETTSSLTLTFWYTLQDDILSFEAERQAVYQQVYRPVYFQLVDVLLHRAQFPSDEEYGFWSSDEREQFRIYRVDISDTLMYVYEMLGAELLSNLYDRLGRLLTSSEEPYSWQHTEALLYGFQSIAETIDVNYSDVVPGLIGLIPRISISNVQLADTVMFTIGALSEWLADHPVMINSVLPLVLHALGNPELSVSSVSTLRRICRECRYDLPPYAANIVAVSQDVLMRQIHRTSQCMWLMQALGFLLSALQVEEILRNLHSLISPYIQQLERLAEEIPNPSNRLAIVHILGLLSNLFTTLDISHHEDDHEGPELRRLPVPQGPNPVVVVLQQVFQLIQRVLSRWLNDAQVVEAVCAIFERSVRTLLDDFAPMVPQLCEMLGRMYSTIPQASALDLTRQLVHIFAHEPAHFPPIEALFLLVTSVTLTLFQQGPRDHPDIVDSFMQLLAQALRRRPDLFLCERLDVRSVFQCAVLALRFPEAPTVRASCGFFTELLPRCGEVESVGRVVQEDGRMLLIAVLEAIGGQASRSLMDCFADILFALNRHCFSLLSMWIREALQPPGFPSARLSPEQRDTFSQQILRERVNRRRVREMVREFTLLCRGLHGTDYTADY

SEQ ID NO: 68 - protein, 908 aa, synthetic construct
  REGION 1..908: note = IPO13 polypeptide fragment
MQAWHFSWQLLQPDRVPEIQYFGASALHIRISRYWSDIPTDQYESLRAQLFTQITRFASGSRIVLTRLCVALASLALSMMPDAWPCAVADMVRLFQAEDSPVDGQGRCLALLELLTVLPEEFQTSRLPQYRRGLVRTSLAVECGAVFPLLEQLLQQPSSPSCVRQRVLRCFSSWVQLEVPLQDCEALIQAAFAALQDSELFDSSVEAIVNAISQPDAQRYVNTLLRLIPLVLGLQEQLRQAVQNGDMETSHGICRIAVALGENHSRALLDQVEHWQSFLALVNMIMFCTGIPGHYPVNETTSSLTLTFWYTLQDDILSFEAERQAVYQQVYRPVYFQLVDVLLHRAQFPSDEEYGFWSSDEREQFRIYRVDISDTLMYVYEMLGAELLSNLYDRLGRLLTSSEEPYSWQHTEALLYGFQSIAETIDVNYSDVVPGLIGLIPRISISNVQLADTVMFTIGALSEWLADHPVMINSVLPLVLHALGNPELSVSSVSTLRRICRECRYDLPPYAANIVAVSQDVLMRQIHRTSQCMWLMQALGFLLSALQVEEILRNLHSLISPYIQQLERLAEEIPNPSNRLAIVHILGLLSNLFTTLDISHHEDDHEGPELRRLPVPQGPNPVVVVLQQVFQLIQRVLSRWLNDAQVVEAVCAIFERSVRTLLDDFAPMVPQLCEMLGRMYSTIPQASALDLTRQLVHIFAHEPAHFPPIEALFLLVTSVTLTLFQQGPRDHPDIVDSFMQLLAQALRRRPDLFLCERLDVRSVFQCAVLALRFPEAPTVRASCGFFTELLPRCGEVESVGRVVQEDGRMLLIAVLEAIGGQASRSLMDCFADILFALNRHCFSLLSMWIREALQPPGFPSARLSPEQRDTFSQQILRERVNRRRVREMVREFTLLCRGLHGTDYTADY

SEQ ID NO: 69 - protein, 872 aa, synthetic construct
  REGION 1..872: note = IPO13 polypeptide fragment
MIPTDQYESLRAQLFTQITRFASGSRIVLTRLCVALASLALSMMPDAWPCAVADMVRLFQAEDSPVDGQGRCLALLELLTVLPEEFQTSRLPQYRRGLVRTSLAVECGAVFPLLEQLLQQPSSPSCVRQRVLRCFSSWVQLEVPLQDCEALIQAAFAALQDSELFDSSVEAIVNAISQPDAQRYVNTLLRLIPLVLGLQEQLRQAVQNGDMETSHGICRIAVALGENHSRALLDQVEHWQSFLALVNMIMFCTGIPGHYPVNETTSSLTLTFWYTLQDDILSFEAERQAVYQQVYRPVYFQLVDVLLHRAQFPSDEEYGFWSSDEREQFRIYRVDISDTLMYVYEMLGAELLSNLYDRLGRLLTSSEEPYSWQHTEALLYGFQSIAETIDVNYSDVVPGLIGLIPRISISNVQLADTVMFTIGALSEWLADHPVMINSVLPLVLHALGNPELSVSSVSTLRRICRECRYDLPPYAANIVAVSQDVLMRQIHRTSQCMWLMQALGFLLSALQVEEILRNLHSLISPYIQQLERLAEEIPNPSNRLAIVHILGLLSNLFTTLDISHHEDDHEGPELRRLPVPQGPNPVVVVLQQVFQLIQRVLSRWLNDAQVVEAVCAIFERSVRTLLDDFAPMVPQLCEMLGRMYSTIPQASALDLTRQLVHIFAHEPAHFPPIEALFLLVTSVTLTLFQQGPRDHPDIVDSFMQLLAQALRRRPDLFLCERLDVRSVFQCAVLALRFPEAPTVRASCGFFTELLPRCGEVESVGRVVQEDGRMLLIAVLEAIGGQASRSLMDCFADILFALNRHCFSLLSMWIREALQPPGFPSARLSPEQRDTFSQQILRERVNRRRVREMVREFTLLCRGLHGTDYTADY

SEQ ID NO: 70 - protein, 826 aa, synthetic construct
  REGION 1..826: note = IPO13 polypeptide fragment
MWPCAVADMVRLFQAEDSPVDGQGRCLALLELLTVLPEEFQTSRLPQYRRGLVRTSLAVECGAVFPLLEQLLQQPSSPSCVRQRVLRCFSSWVQLEVPLQDCEALIQAAFAALQDSELFDSSVEAIVNAISQPDAQRYVNTLLRLIPLVLGLQEQLRQAVQNGDMETSHGICRIAVALGENHSRALLDQVEHWQSFLALVNMIMFCTGIPGHYPVNETTSSLTLTFWYTLQDDILSFEAERQAVYQQVYRPVYFQLVDVLLHRAQFPSDEEYGFWSSDEREQFRIYRVDISDTLMYVYEMLGAELLSNLYDRLGRLLTSSEEPYSWQHTEALLYGFQSIAETIDVNYSDVVPGLIGLIPRISISNVQLADTVMFTIGALSEWLADHPVMINSVLPLVLHALGNPELSVSSVSTLRRICRECRYDLPPYAANIVAVSQDVLMRQIHRTSQCMWLMQALGFLLSALQVEEILRNLHSLISPYIQQLERLAEEIPNPSNRLAIVHILGLLSNLFTTLDISHHEDDHEGPELRRLPVPQGPNPVVVVLQQVFQLIQRVLSRWLNDAQVVEAVCAIFERSVRTLLDDFAPMVPQLCEMLGRMYSTIPQASALDLTRQLVHIFAHEPAHFPPIEALFLLVTSVTLTLFQQGPRDHPDIVDSFMQLLAQALRRRPDLFLCERLDVRSVFQCAVLALRFPEAPTVRASCGFFTELLPRCGEVESVGRVVQEDGRMLLIAVLEAIGGQASRSLMDCFADILFALNRHCFSLLSMWIREALQPPGFPSARLSPEQRDTFSQQILRERVNRRRVREMVREFTLLCRGLHGTDYTADY

SEQ ID NO: 71 - protein, 783 aa, synthetic construct
  REGION 1..783: note = IPO13 polypeptide fragment
MLPQYRRGLVRTSLAVECGAVFPLLEQLLQQPSSPSCVRQRVLRCFSSWVQLEVPLQDCEALIQAAFAALQDSELFDSSVEAIVNAISQPDAQRYVNTLLRLIPLVLGLQEQLRQAVQNGDMETSHGICRIAVALGENHSRALLDQVEHWQSFLALVNMIMFCTGIPGHYPVNETTSSLTLTFWYTLQDDILSFEAERQAVYQQVYRPVYFQLVDVLLHRAQFPSDEEYGFWSSDEREQFRIYRVDISDTLMYVYEMLGAELLSNLYDRLGRLLTSSEEPYSWQHTEALLYGFQSIAETIDVNYSDVVPGLIGLIPRISISNVQLADTVMFTIGALSEWLADHPVMINSVLPLVLHALGNPELSVSSVSTLRRICRECRYDLPPYAANIVAVSQDVLMRQIHRTSQCMWLMQALGFLLSALQVEEILRNLHSLISPYIQQLERLAEEIPNPSNRLAIVHILGLLSNLFTTLDISHHEDDHEGPELRRLPVPQGPNPVVVVLQQVFQLIQRVLSRWLNDAQVVEAVCAIFERSVRTLLDDFAPMVPQLCEMLGRMYSTIPQASALDLTRQLVHIFAHEPAHFPPIEALFLLVTSVTLTLFQQGPRDHPDIVDSFMQLLAQALRRRPDLFLCERLDVRSVFQCAVLALRFPEAPTVRASCGFFTELLPRCGEVESVGRVVQEDGRMLLIAVLEAIGGQASRSLMDCFADILFALNRHCFSLLSMWIREALQPPGFPSARLSPEQRDTFSQQILRERVNRRRVREMVREFTLLCRGLHGTDYTADY

SEQ ID NO: 72 - protein, 732 aa, synthetic construct
  REGION 1..732: note = IPO13 polypeptide fragment
MEVPLQDCEALIQAAFAALQDSELFDSSVEAIVNAISQPDAQRYVNTLLRLIPLVLGLQEQLRQAVQNGDMETSHGICRIAVALGENHSRALLDQVEHWQSFLALVNMIMFCTGIPGHYPVNETTSSLTLTFWYTLQDDILSFEAERQAVYQQVYRPVYFQLVDVLLHRAQFPSDEEYGFWSSDEREQFRIYRVDISDTLMYVYEMLGAELLSNLYDRLGRLLTSSEEPYSWQHTEALLYGFQSIAETIDVNYSDVVPGLIGLIPRISISNVQLADTVMFTIGALSEWLADHPVMINSVLPLVLHALGNPELSVSSVSTLRRICRECRYDLPPYAANIVAVSQDVLMRQIHRTSQCMWLMQALGFLLSALQVEEILRNLHSLISPYIQQLERLAEEIPNPSNRLAIVHILGLLSNLFTTLDISHHEDDHEGPELRRLPVPQGPNPVVVVLQQVFQLIQRVLSRWLNDAQVVEAVCAIFERSVRTLLDDFAPMVPQLCEMLGRMYSTIPQASALDLTRQLVHIFAHEPAHFPPIEALFLLVTSVTLTLFQQGPRDHPDIVDSFMQLLAQALRRRPDLFLCERLDVRSVFQCAVLALRFPEAPTVRASCGFFTELLPRCGEVESVGRVVQEDGRMLLIAVLEAIGGQASRSLMDCFADILFALNRHCFSLLSMWIREALQPPGFPSARLSPEQRDTFSQQILRERVNRRRVREMVREFTLLCRGLHGTDYTADY

SEQ ID NO: 73 - protein, 488 aa, synthetic construct
  REGION 1..488: note = IPO13 polypeptide fragment
MAETIDVNYSDVVPGLIGLIPRISISNVQLADTVMFTIGALSEWLADHPVMINSVLPLVLHALGNPELSVSSVSTLRRICRECRYDLPPYAANIVAVSQDVLMRQIHRTSQCMWLMQALGFLLSALQVEEILRNLHSLISPYIQQLERLAEEIPNPSNRLAIVHILGLLSNLFTTLDISHHEDDHEGPELRRLPVPQGPNPVVVVLQQVFQLIQRVLSRWLNDAQVVEAVCAIFERSVRTLLDDFAPMVPQLCEMLGRMYSTIPQASALDLTRQLVHIFAHEPAHFPPIEALFLLVTSVTLTLFQQGPRDHPDIVDSFMQLLAQALRRRPDLFLCERLDVRSVFQCAVLALRFPEAPTVRASCGFFTELLPRCGEVESVGRVVQEDGRMLLIAVLEAIGGQASRSLMDCFADILFALNRHCFSLLSMWIREALQPPGFPSARLSPEQRDTFSQQILRERVNRRRVREMVREFTLLCRGLHGTDYTADY

SEQ ID NO: 74 - protein, 933 aa, synthetic construct
  REGION 1..933: note = IPO13 polypeptide fragment
MERREEQPGAAGAGAAPALDFTVENVERALHQLYYDPNIENRNLAQRWLMQAQVSPQAWHFSWQLLQPDRVPEIQYFGASALHIRISRYWSDIPTDQYESLRAQLFTQITRFASGSRIVLTRLCVALASLALSMMPDAWPCAVADMVRLFQAEDSPVDGQGRCLALLELLTVLPEEFQTSRLPQYRRGLVRTSLAVECGAVFPLLEQLLQQPSSPSCVRQRVLRCFSSWVQLEVPLQDCEALIQAAFAALQDSELFDSSVEAIVNAISQPDAQRYVNTLLRLIPLVLGLQEQLRQAVQNGDMETSHGICRIAVALGENHSRALLDQVEHWQSFLALVNMIMFCTGIPGHYPVNETTSSLTLTFWYTLQDDILSFEAERQAVYQQVYRPVYFQLVDVLLHRAQFPSDEEYGFWSSDEREQFRIYRVDISDTLMYVYEMLGAELLSNLYDRLGRLLTSSEEPYSWQHTEALLYGFQSIAETIDVNYSDVVPGLIGLIPRISISNVQLADTVMFTIGALSEWLADHPVMINSVLPLVLHALGNPELSVSSVSTLRRICRECRYDLPPYAANIVAVSQDVLMRQIHRTSQCMWLMQALGFLLSALQVEEILRNLHSLISPYIQQLERLAEEIPNPSNRLAIVHILGLLSNLFTTLDISHHEDDHEGPELRRLPVPQGPNPVVVVLQQVFQLIQRVLSRWLNDAQVVEAVCAIFERSVRTLLDDFAPMVPQLCEMLGRMYSTIPQASALDLTRQLVHIFAHEPAHFPPIEALFLLVTSVTLTLFQQGPRDHPDIVDSFMQLLAQALRRRPDLFLCERLDVRSVFQCAVLALRFPEAPTVRASCGFFTELLPRCGEVESVGRVVQEDGRMLLIAVLEAIGGQASRSLMDCFADILFALNRHCFSLLSMWIREALQPPGFPSARLSPEQRDTFSQQILRE

SEQ ID NO: 75 - protein, 896 aa, synthetic construct
  REGION 1..896: note = IPO13 polypeptide fragment
MERREEQPGAAGAGAAPALDFTVENVERALHQLYYDPNIENRNLAQRWLMQAQVSPQAWHFSWQLLQPDRVPEIQYFGASALHIRISRYWSDIPTDQYESLRAQLFTQITRFASGSRIVLTRLCVALASLALSMMPDAWPCAVADMVRLFQAEDSPVDGQGRCLALLELLTVLPEEFQTSRLPQYRRGLVRTSLAVECGAVFPLLEQLLQQPSSPSCVRQRVLRCFSSWVQLEVPLQDCEALIQAAFAALQDSELFDSSVEAIVNAISQPDAQRYVNTLLRLIPLVLGLQEQLRQAVQNGDMETSHGICRIAVALGENHSRALLDQVEHWQSFLALVNMIMFCTGIPGHYPVNETTSSLTLTFWYTLQDDILSFEAERQAVYQQVYRPVYFQLVDVLLHRAQFPSDEEYGFWSSDEREQFRIYRVDISDTLMYVYEMLGAELLSNLYDRLGRLLTSSEEPYSWQHTEALLYGFQSIAETIDVNYSDVVPGLIGLIPRISISNVQLADTVMFTIGALSEWLADHPVMINSVLPLVLHALGNPELSVSSVSTLRRICRECRYDLPPYAANIVAVSQDVLMRQIHRTSQCMWLMQALGFLLSALQVEEILRNLHSLISPYIQQLERLAEEIPNPSNRLAIVHILGLLSNLFTTLDISHHEDDHEGPELRRLPVPQGPNPVVVVLQQVFQLIQRVLSRWLNDAQVVEAVCAIFERSVRTLLDDFAPMVPQLCEMLGRMYSTIPQASALDLTRQLVHIFAHEPAHFPPIEALFLLVTSVTLTLFQQGPRDHPDIVDSFMQLLAQALRRRPDLFLCERLDVRSVFQCAVLALRFPEAPTVRASCGFFTELLPRCGEVESVGRVVQEDGRMLLIAVLEAIGGQASRSLMDCFADILFALNRHC

SEQ ID NO: 76 - protein, 476 aa, synthetic construct
  REGION 1..476: note = IPO13 polypeptide fragment
MERREEQPGAAGAGAAPALDFTVENVERALHQLYYDPNIENRNLAQRWLMQAQVSPQAWHFSWQLLQPDRVPEIQYFGASALHIRISRYWSDIPTDQYESLRAQLFTQITRFASGSRIVLTRLCVALASLALSMMPDAWPCAVADMVRLFQAEDSPVDGQGRCLALLELLTVLPEEFQTSRLPQYRRGLVRTSLAVECGAVFPLLEQLLQQPSSPSCVRQRVLRCFSSWVQLEVPLQDCEALIQAAFAALQDSELFDSSVEAIVNAISQPDAQRYVNTLLRLIPLVLGLQEQLRQAVQNGDMETSHGICRIAVALGENHSRALLDQVEHWQSFLALVNMIMFCTGIPGHYPVNETTSSLTLTFWYTLQDDILSFEAERQAVYQQVYRPVYFQLVDVLLHRAQFPSDEEYGFWSSDEREQFRIYRVDISDTLMYVYEMLGAELLSNLYDRLGRLLTSSEEPYSWQHTEALLYGFQSI

SEQ ID NO: 77 - protein, 523 aa, synthetic construct
  REGION 1..523: note = IPO13 polypeptide fragment
MERREEQPGAAGAGAAPALDFTVENVERALHQLYYDPNIENRNLAQRWLMQAQVSPQAWHFSWQLLQPDRVPEIQYFGASALHIRISRYWSDIPTDQYESLRAQLFTQITRFASGSRIVLTRLCVALASLALSMMPDAWPCAVADMVRLFQAEDSPVDGQGRCLALLELLTVLPEEFQTSRLPQYRRGLVRTSLAVECGAVFPLLEQLLQQPSSPSCVRQRVLRCFSSWVQLEVPLQDCEALIQAAFAALQDSELFDSSVEAIVNAISQPDAQRYVNTLLRLIPLVLGLQEQLRQAVQNGDMETSHGICRIAVALGENHSRALLDQVEHWQSFLALVNMIMFCTGIPGHYPVNETTSSLTLTFWYTLQDDILSFEAERQAVYQQVYRPVYFQLVDVLLHRAQFPSDEEYGFWSSDEREQFRIYRVDISDTLMYVYEMLGAELLSNLYDRLGRLLTSSEEPYSWQHTEALLYGFQSIAETIDVNYSDVVPGLIGLIPRISISNVQLADTVMFTIGALSEWLADH

SEQ ID NO: 78 - protein, 206 aa, synthetic construct
  REGION 1..206: note = wild type C-terminal fragment of human TDP-43 from amino acid 207-414 (TDP-CTF) polypeptide
REFFSQYGDVMDVFIPKPFRAFAFVTFADDQIAQSLCGEDLIIKGISVHISNAEPKHNSNRQLERSGRFGGNPGGFGNQGGFGNSRGGGAGLGNNQGSNMGGGMNFGAFSINPAMMAAAQAALQSSWGMMGMLASQQNQSGPSGNNQNQGNMQREPNQAFGSGNNSYSGSNSGAAIGWGSASNAGSGSGFNGGFGSSMDSKSSGWM

SEQ ID NO: 79 - protein, 206 aa, synthetic construct
  REGION 1..206: note = VLIM-F variant TDP-CTF polypeptide having all V, L, I, and M amino acid residues mutated to F
REFFSQYGDVMDVFIPKPFRAFAFVTFADDQIAQSLCGEDLIIKGISVHISNAEPKHNSNRQFERSGRFGGNPGGFGNQGGFGNSRGGGAGFGNNQGSNFGGGFNFGAFSFNPAMMAAAQAALQSSWGMMGMLASQQNQSGPSGNNQNQGNFQREPNQAFGSGNNSYSGSNSGAAFGWGSASNAGSGSGFNGGFGSSFDSKSSGWF

SEQ ID NO: 80 - protein, 12 aa, synthetic construct
  REGION 1..12: note = linker polypeptide
GGGSGGGSGGGS